European Patent Specification EP 3 337 889 B1, published April 26, 2023. Title: Methods for Fermentative Production of Massoia Lactone. Applicant: Temasek Life Sciences Laboratory Limited. The sequence listing filed with the application follows.

SEQUENCE LISTING (10 sequences)

SEQ ID NO: 1 - DNA, 666 bp, Aureobasidium melanogenum strain W5-2
  misc_feature (36)..(36): n is a, c, g, or t
agcgtcccgccaaagcaacaagtagttttaacaacnaagggttcttggtcatttagaggaagtaaaagtcgtaaacaaggcttccgtaaggtgaacctgcggaaggatcattaaagagtaagggtgctcagcgcccgacctccaaccctttgttgttaaaactaccttgttgctttggcgggaccgctcggtctcgagccgctggggattcgtcccaggcgagcgcccgccagagttaaaccaaactcttgttatttaaccggtcgtctgagttaaaattttgaataaatcaaaactttcaacaacggatctcttggttctcgcatcgatgaagaacgcagcgaaatgcgataagtaatgtgaattgcagaattcagtgaatcatcgaatctttgaacgcacattgcgccccttggtattccgaggggcatgcctgttcgagcgtcattacaccactcaagctatgcttggtattgggtgccgtccttagttgggcgcgccttaaagacctcggcgaggcctcaccggctttaggcgtagtagaatttattcgaacgtctgtcaaaggagaggacttctgccgactgaaaccttttatttttctaggttgacctcggatcaggtagggatacccgctgaacttaagcatatcaataagcggaggaa

SEQ ID NO: 2 - DNA, 1014 bp, Aureobasidium species
atgcctgtcaacgtcggtattaacggcttcggtcgcattggtcgcattgtcttccgcaatgccatcgagctcgacaacgtccacgtcgttgccgtcaacgaccccttcattgagcccgagtacgctgcctacatgctcaagtacgactccgtccacggccagttcaagggtaccattgaggtctccggcaaggacctgatcgtcaacggcaagaaggtcaccttctacaccgagagagaccccgccaacatcccctgggctgagactggcgcctactacgtcgtcgagtccaccggtgtcttcaccaccaccgagaaggcctccgctcacttgaagggtggcgccaagaaggtcgtcatctctgctccctccgctgacgcccccatgttcgtcatgggtgtcaacgagaagagctacaagtccgacatccaggtcctgtccaacgcctcttgcaccaccaactgccttgctcccctcgccaaggtcatcaacgacaagttcggtatcgttgagggtctcatgaccaccatccactcctacaccgccacccagaagaccgtcgacggtccttccggcaaggactggcgcggtggccgtgctgctgcccagaacatcatccccagcagcactggtgccgccaaggctgtcggcaaggtcattcctcagctcaacggcaagctgaccggtatgtccatgcgtgtccccaccgccaacgtctccgttgtcgaccttactgcccgtctcgagaagggtgcctcttacgacaccatcaagaaggccatcaaggaggcctccgagggtgagcttaagggcattctcggctacaccgaggacgacattgtctcctccgacatgtgcggtgccaacgagtcctccatcttcgacgccaaggccggtatctcgctcaacgacaacttcgtcaagcttgtctcctggtacgacaacgagtggggttactcccgccgtgtcctcgacctcctggcttacattgccaaggtcgacggtaacgcataa

SEQ ID NO: 3 - DNA, 19 bp, Artificial Sequence
  oligonucleotide primer
tccgtaggtgaacctgcgg

SEQ ID NO: 4 - DNA, 20 bp, Artificial Sequence
  oligonucleotide primer
tcctccgcttattgatatgc

SEQ ID NO: 5 - DNA, 35683 bp, Aureobasidium pullulans strain BP-1938
  CDS (506)..(35485)
cgatggcaactgttgccaacaaagcggaaaatttctctatgcggaggtgtgttacgaatctgcctaacttttgcctcatccactgacgactgactaatcacagggaggttagtgttcgctgccgagggcgccatgtcaggcgtcgcccggcagagttgatcatgcaaattcgaagtgagcaccgatcagatgagtcaagtcaatatgcattgtcttatagccagacgatatgcgcgccacaacgattcttgctgacatcacccatatacagtcataagtgtagttcgcttacggagctcacatgaccgcaatgtctatcagagtaagcatgtctgtcgtggctgacgctgctctaacaatgatgcgtgaagcatcagtcaatcagcaagcgaggaatacttctgccacattgaccagactatcaaccctctgacatcgagcaacagcgacagcaaacgtttgactacaacaacagccaccgtatagcaacattcaacaaacaaagatgtcgcgaatgccacagggcgcagcaagacgcaacgactgtgtctcggagcaccaaggcactaccgatctggaggatattgtgcgattctgggaacgacacttagacggtgtgaatgcatctgcattccctgctctgtcatctagcttggttgtacctaaacccaaattgcagacagagcatcgcatcagcctcggaaccgccgtgtctgatcagtggtcagatgcagtcatctgtcgagctgcacttgctgtcattttggcccgttatacgcacgctactgaagcgctctacggcattgtggtcgagcagccttcagtctccaatgcccagaaacgatccgccgatgatgcatcctccattgttgtaccgattcgtgtgcaatgtgcatctggtcaatttgggaacgatattttggctgcaattgctactcacgacgcttcttgtcgtagcctcagcgcgatcggcctggatggcattcgctgtcttgatgatgctaaaactgtggctcggggattacagactgtattgactgtaaccagcaggaagtcggtggacgcatcaagcccaaacattctcgacttggagaacatcgcatcttctcacggtcgagctctcatgatagaatgtcaaatgagcaccacctcggcatgcttgcgtgcacagtacgacgcgggcatcttgcgtaatgaacaggtagttcgtcttctcaaacagctcgcgctttcgatccagcactttcgaggtaacgctgccaacgacctgctacgcgacttctgctttatctcgccaggcgaagagatggaaattgcatactggaatcgtcgaagcattcgcacaaatgaggtttgtatccatgatgtgatctttaagagggcgacctacatgccgactgatacggcggtttccgcctgggatggggagtggacatacgcagatctagatgtcgtatcttcatgtcttgccgattacgttcggtccttggatctgaggtctggacaagccataccactatgcttcgagaagtcaagaaacaccatcgccgctatggtggccgttctcaaagctggtcatccgttttgcctgattgacccgtctactccatctgcgagaatcactcagatgtgcgagcagatgtccgctaccgtcgctttcgcttcgagagcactttgtagcatcatgcaagcaggagtctctagatgtattgcagttgatgacgatctctttcaatccttgtcatcagtcatcgggtgtccacagatgtccatgacgagaccccaggaccttgcctatgtcatatttacatccggaagtactggaatcccgaagggcagcatgatcgagcatcgaggttttgcaagctgcgcacttgaattcggacctcaattgttaatcgatcgcaacacgcgtgcattacagttcgcctctcacgcttttggcgcatgcttgttagaggttctggtgacgcttatgcttggaggttgtgtatgcgtcccgtccgaaaacgatcgcttgaacaacctgtcaggtttcattgaacaaagcggcgtgaactggaccctatttacgccttcttttattggagctctcacgcccgagactattcgtggggtgcacactgtcgtgctgggtggagagccaatgacaccattcatcagagacgtatgggcatcaaaagtgcaactcttgtccatatatggacaaagtgagagctcgactgtgtgtagtgtggttaaaatcaagcctgataccaccgatctgagtagcctgggccacgctataggagctcgcttctggatcgttgatgctgaaaatccgagtcgattggcaccaatcggctgcatcggcgagctcatggtagagagtcctggaattgcacgcgaatacctatctgctcaagaagcacagatgtccccattcataacgaagacacctgcttggtatcctatgaagcagcgttgcagtcctgtcaagttctacatgaccggcgatcttgcttgttatggacgtgatggcaccgtcatgaatcttggacgcaaagattcgcaagtcaagatccgaggccaacgcgtggagcttggcgatgtggagactaatctgcgatcagtcttacctaaacacatcatacctgttgtcgaggcgattgattcgatccatgcatccggaagcaaatttctggttgcgatcctgattggcgcaaaccatggaatgaaaaatgaattcgatacagagccaagacgtgaagtctctatactggatgaaaccgcggtgatccgtataaggaagagtatgcaggatcttgttccatcttactgcatacccacacagtatatctgcatggaacgactcctgaccacgacaacagggaaggcggatcgcaagagactacgcgcgatttgcgtggaccttctcaagccttcaaggagagcaatggtaccagaatcttcggacgggcccacgctaaaactcacggcaggacaagttttggatgaggcatggcatcgatacctgcgttttgattctgttctcgatggttctaagtcgaagttctttgatctgaatggagactccatcacagcgatcaagatagcaaatgcggcgaggaaacacggggtaatgctcaaagtagcagacattcttgctaatcctactctcgccgacctgagagctcaatttcagattgatttcacacctcaaaactccatacttcgcacctcgtaccgtggaccaatccaacaatcctttgcgcaaaacaggttgtggtttctggaccagctgaacgttggcgcgtcatggtacatagtaccagtcgcggtgcgcttgcaaggaacagtccatgtcgacgcgcttgtcaccgcactatgtgccctggaacaacgtcatgaaacgttgcgtacgacctttgaagaatccgatggcgagggcatacaacggattcagccaagtgggcttgagcagcttaggttgatcgacgtggattgcgtggactctagggactaccagcgagtattggaagaagagcagacgactcccttcgagctgagccgcgagcctggatggagggtagcgctgctgcgtctgggagatgacgaccacgtcctctccatcgtcatgcatcacatcatctccgacggttggtctgtggacgtgctgcgccacgagctaggtcagttctactcggccgcgctccgggggcaggacccgttgtcgcagataagtcctctgccgatccagtatcgtgacttcgctctctggcagagacaagacgagcaagttgcggagcatcagcgccagctggagcattggacagagcagttggcagacagttcacccgccgagttgttgagcgaccacccgaggccatcgattctttctggccaggcgggcgctattcccgtcaatgttcaaggctctctgtatcaggcgcttcgggcgttctgccgcgctcaccaggtcacctctttcgtagtcctgctcacggcgttccgcatagcacactatcgtctgacgggtgcggaggacgcaaccattggaactcccattgcaaatcgcaaccggccagagctcgagaacatgatcggtttcttcgtcaatacacaatgcatgcgcatcgtcattggcagtgacgacacatttgaagggctggtgcagcaagtacgctcgataactgcagctgcccacgagaaccaggacgttccattcgagcgcatcgtgtcagcactgcttcccggttctagagacacatcacgcaatcctctggttcagctcatgtttgctgtccactcgcaaagaaaccttggtcagatcagtctagaaggcctgcagggtgaattgctgggagtggcatcgccaacgagattcgatgtagagttccacctcttccaagaggagaatatgctaagcggaagggtgctgttttcagacgatcttttcgagcagaagactatgcaaggcatggtcgacgtgttccaggaagtgctcagccggggccttgagcagccccagatacctctggcgaccctcccgctcacgcacggactggaggagctcaggaccatgggtcttctcgacgtggagaagacagactaccctcgagagtcgagcgtggtggacgtgttccgtgagcaagcggctgcctgctccgaggcgattgcggtcaaagactcgtcggcgcagctcacctactcggagctcgatcgacagtcggacgagcttgccggctggctgcgccagcaacgtcttcctgcggagtcgttggttgcagtgctggcacccaggtcgtgccagaccattgtcgcgttcctgggcatcctcaaggcgaatctggcatacctgccgctagacgtcaacgtgcccgctactcgcctcgagtcgatactgtctgccgtcggcggccggaagctggtcttgcttggagctgacgtggccgaccctggccttcgcctggcggatgtggagctcgtgcggatcggcgacacactcggccgctgtgtacccggggcgcccggcgacaacgaggcacctgtggtgcagccttctgccacaagccttgcctacgtcatcttcacttccggctcgaccggcaagccgaagggtgtcatggtcgagcaccggggtgtagtgcgacttgtcaagcagagcaatgttgtctaccatctcccgtccacatctcgcgtggcccacctgtcgaatctcgcctttgatgcctcggcgtgggagatctatgcggcactgcttaatggcggtacactcatctgcattgactatttcacaactctagactgctctgctctcggcgccaaattcatcaaggagaagatcgtcgcgaccatgattccgccagcgcttctgaagcaatgtctggcgatcttcccgaccgctcttagtgaactggtcctgctgtttgctgccggagatcgattcagcagtggcgatgccgtcgaagtgcagcgccacaccaaaggcgctgtttgtaacgcgtacggaccgacagaaaacaccattcttagtacgatctacgaagtcaagcagaatgagaacttcccgaacggtgtgcctatcggccgcgctgtgagcaactcaggggcatatgtcatggacccgcagcagcaactggtgcctctcggggtgatgggcgagctcgtcgtcaccggcgacggcctggcccgtggttacaccgacccgtcactggatgcggaccgctttgtgcaggtctccgtcaacgggcagctcgtgagagcgtaccgaacaggcgatcgcgtgcgctgcaggccttgcgatggccagatcgagttctttggacgtatggaccggcaagtcaagatccgaggacatcgcatcgagctcgcagaggtagagcatgcggtgcttggcttggaagacgtgcaagacgctgccgttatcgcatttgacaatgtggacagcgaagagccagaaatggttgggtttgtcactattaccgaagacaatcctgtccgtgaggacgaaaccagcggtcaagtagaagactgggcgaaccacttcgagataagtacctacaccgatatcgcggcgatcgatcagggtagcattggaagtgactttgtaggttggacttctatgtacgacggaagcgagatcgacaaggcagagatgcaagaatggcttgccgataccatggcctctatgctcgacgggcaggcgccgggcaatgtgttagagataggtacaggcactggcatggtcctcttcaatctcggcgacggactgcagagctatgtcggcctcgaaccatcaagatcggcggccgcttttgtcaaccagacgattaagtcgctccccacccttgctggcaacgctgaagtacacattggcactgcgaccgacgtggcccgtctagatggcctccgccccgacttagtggtagtcaattcggtagtccagtacttcccatcaccagagtacctaatggaagtcgtggaggctcttgcacgtctgccgggcgtcgagcgaattttcttcggagacgtacgttcgtacgccatcaacagagatttcctggctgccagagctctacacgaacttggcgacagagcgactaagcacgagattcggcgaaagatgctagagatggaagaacgcgaagaggagctgctcgtcgacccagctttcttcaccatgttgaccagcagtctccctggcctgattcagcatgtcgagatcttgccgaagctgatgagagccactaatgagctcagcgcgtatcgatacactgctgtagtacacgtgtgccgtgccggtcaagagcctcgttccgtgcatacgatcgacgacgatgcctgggtgaatcttggagcttctcggttgagtcgccctaccctttcaagccttttgcaaacttccgagggcgcatcggccgtcgcagtaagcaatattccttacagcaagaccatcacagagcgagcgctcgttagtgcgctcgatgaggatgatatgcaagactcatcggactggctgctggccgtgcgcgagacaggcagatcttgttcctccttctccgcaacagaccttgtcgagcttgctcgagagacgggctggcgtgtggagctcagctgggcacgacagtactcacagaaaggcgcactcgatgctgtcttccacagacaccctgtttccgctgggagcgggcgtgtcatgttccagtttccagttgagaccgaagatcgaccgcacatctcacgcacgaaccgacctttacagcgattgcagaagaagcgaaccgagacacatgttcatgagcagttgcgggctttgcttccacgatacatggttcctacgcggattgtggcgcttgataagctgcccgtcaatgcaaacggcaaggttgatcgtcaacagctcgctaggacagcccaggttctcccagcgagcaaggcgccgtctgcatgcgtggccccacgcaacgaattggaaatgacactgtgtgaagagttctcgcaggttcttggcgtcgaggtcggcattactgacaatttcttccacctgggtggccactctctcatggcaacaaagttcgccgctcgtatcagccgccggctgaatgctatcgtttcggtcaagaatgtcttcgaccaccccgtacctatggatcttgcagcgacaatccaagaaggctcaaagcttcatactccaatccctcgcacggcttacagcggtcctgtcgaacagtctttcgcacaaggacgtctttggttccttgaccaattcaatcctagctcgattgggtatgtgatgcctttcgctgcgcgtcttcatggtcaactacaaatcgaagcgctcacagcagcattgttcgctttggaacagcgacatgagatcctgcgaacaacgttggacgcacacgatggtgtaggcatgcagatcgttcacgcggaacatccgcaacagttgagaatcattgatgtgtcagcaaaggcgtcgagcagttatgctcagacactgcgtgacgagcaggcgtcacctttcgacctaagcaaggaaccaggttggagagtctcgttgctgcagctcagtgagatagattatgttctttccattgtaatgcatcacaccatctatgacggttggtctctcgacgtactccggcgggagctaagtcagttttatgccgctgccatccgtggtcgagaacctctatcgacaatcgagccattgcctatccaataccgcgacttttctgtctggcaaaagcaggaagaccaagtcgcagagcatcgacgacagctccattattggatagagcagctagatggcagctctcctgctgagttcctaaacgataaaccacggcctacgttgctttctggcaaggcaggagttgtggaaattgctgtgaagggcactgtatatcaacgtctgctagagttctgcaggcttcatcaggtcacctcgttcatggtgctgcttgcggcattccgagcgacacactatcgtctgacaggcacagaggacgcgactgtcggaacacccatcgccaatcgcaatcgacctgagctggagaacatgattggattgttcgtgaatactcagtgtatacgcctcaagatcgaggacaatgatactctcgaggagctagtacagcacgttcgtgccacgatcacagcatcaatctcgaaccaggatgtaccctttgaacaggtagtgtctgcattgctaccaggatcacgcgacacctctaggaacccactagttcagctgacttttgcggtgcattctcagcgaaatttggctgacattcagctagaaaacgtggagaccaatgctatgccaatttgcccctcgacacgtttcgacgctgaattccacctcttccaagaggagaatatgctaagcggaagggtgctgttttcagacgatcttttcgagcagaagactatgcaaggcatggtcgacgtgttccaggaagtgctcagccggggccttgagcagccccagatacctctggcgaccctcccgctcacgcacggactggaggagctcaggaccatgggtcttctcgacgtggagaagacagactaccctcgagagtcgagcgtggtggacgtgttccgtgagcaagcggctgcctgctccgaggcgattgcggtcaaagactcgtcggcgcagctcacctactcggagctcgatcgacagtcggacgagcttgccggctggctgcgccagcaacgtcttcctgcggagtcgttggttgcagtgctggcacccaggtcgtgccagaccattgtcgcgttcctgggcatcctcaaggcgaatctggcatacctgccgctagacgtcaacgtgcccgctactcgcctcgagtcgatactgtctgccgtcggcggccggaagctggtcttgcttggagctgacgtggccgaccctggccttcgcctggcggatgtggagctcgtgcggatcggcgacacactcggccgctgtgtacccggggcgcccggcgacaatgaggcacctgtggtgcagccttctgccacaagccttgcctacgtcatcttcacttccggctcgaccggcaagccgaagggtgtcatggtcgagcaccgtagtatcgtccgcttgatgaggcacagcaatgtctcgagtcgccttctgctacatccccgcatgacccacctgtcgaatctcgccttcgatgcgtcggtgtgggagattttcttgacgctgctcaacggtggaacattgatttgtattgactacctctcgtcactagactgtcgtgctcttggggtaagtatcctggaacaccaggttgacgcatcggtacttcctcctgctttgctcaaacaatgcctagcaaatgtccctgaggcacttgcgagcctgcaagtgctcttgtccgctggagatcgactcgacagtcgtgatgctatagagagttgcgcactcgtgcgcggaagtgtctacaatgggtatggtcccacggagaatggcatccagagcacaatctatgaagtcaaagcggacgctgagtttgtcaatggtgtgcctatcggccgcgctgtgagcaactcaggggcatatgtcatggacccgcagcagcaactggtgcctctcggggtgatgggcgagctcgtcgtcaccggcgacggcctggcccgtggttacaccgacccgtcactggatgcggaccgctttgtgcaggtctccgtcaacgggcagctcgtgagagcgtaccgaacaggcgatcgcgtgcgctgcaggccttgcgatggccagatcgagttctttggacgtatggaccggcaagtcaagatccgaggacatcgcatcgagctcgcagaggtagagcatgcggtgcttggcttggaagacgtgcaagacgctgccgttctcatagctcaaacagccgaaaatgaagagctagttggcttcttcacgcttcgacaaacccaggctgtgcagtcaaatggtgccgctggtgttgtgccagagcacagcgactccgagctggcgcaatcctgctcttgcactcaaacggagcgtcgagtccgcaacagattgcaatcctgtcttcctcgctacatggttccgtcgcgaatggtccttttggatcgactgcctgtcaaccccaatggtaaagttgatcgacaagagctcacgaggcgcgctcaggatctcccaataagcgagtcatccccagtgcacgtcaaaccgcgtactgaactggaaaggtcgctgtgcgaggagttcgccgatgttataggtttggaagtcggcgttaccgataatttcttcgacctaggcgggcactctctcatggcgatgaaactcgcagctcgcatcagccgtcgttcgaatgcacatatatcagtcaaggacattttcgaccacccgctgattgcagatctcgcaatgaaaattcgggaaggctccgatctgcacactccaattccccacaggatgtacgttggacctatccagctatcattcgcacagggacgcttgtggttcctcgaccaattgaatttgggcgcatcgtggtacgtcatgccacttgctatgcgcctccaaggctcgctccagctcgacgcgttagagactgcactgtttgctatcgagcagcgacacgaaaccttacggatgacatttgcagaacaagacggagtagctgtacaagtagtgcatgcagcccactacaaacacatcaagatgatcgacaaaccacttagacagaagattgacgtcctgaagatgctggaagaagaacggacgactcccttcgagctgagccgcgagcctggatggagggtagcgctgctgcgtctgggagatgacgaccacgtcctctccatcgtcatgcatcacatcatctccgacggttggtctgtggacgtgctgcgccacgagctaggtcagttctactcggccgcgctccgggggcaggacccgttgtcgcagataagtcctctgccgatccagtatcgtgacttcgctctctggcagagacaagacgagcaagttgcggagcatcagcgccagctggagcattggacagagcagttggcagacagttcacccgccgagttgttgagcgaccacccgaggccatcgattctttctggccaggcgggcgctattcccgtcaatgttcaaggctctctgtatcaggcgcttcgggcgttctgccgcgctcaccaggtcacctctttcgtagtcctgctcacggcgttccgcatagcacactatcgtctgacgggtgcggaggacgcaaccattggaactcccattgcaaatcgcaaccggccagagctcgagaacatgatcggtttcttcgtcaatacacaatgcatgcgcatcgtcattggcagtgacgacacatttgaagggctggtgcagcaagtacgctcgataactgcagctgcccacgagaaccaggacgttccattcgagcgcatcgtgtcagcactgcttcccggttctagagacacatcacgcaatcctctggttcagctcatgtttgctgtccactcgcaaagaaaccttggtcagatcagtctagaaggcctgcagggtgaattgctgggagtggcagcgactacgagattcgatgtagagttccatctcttccaagatgacgacaagctcagcggcaacgtgctcttcgcgaccgagctcttcgagcagaagactatgcaaggcatggtcgacgtgttccaggaagtgctcagccggggccttgagcagccccagatacctctggcgaccctcccgctcacgcacggactggaggagctcaggaccatgggtcttctcgacgtggagaagacagactaccctcgagagtcgagcgtggtggacgtgttccgtgagcaagcggctgcctgctccgaggcgattgcggtcaaagactcgtcggcgcagctcacctactcggagctcgatcgacagtcggacgagcttgccggctggctgcgccagcaacgtcttcctgcggagtcgttggttgcagtgctggcacccaggtcgtgccagaccattgtcgcgttcctgggcatcctcaaggcgaatctggcatacctgccgctagacgtcaacgtgcccgctactcgcctcgagtcgatactgtctgccgtcggcggccggaagctggtcttgcttggagctgacgtggccgaccctggccttcgcctggcggatgtggagctcgtgcggatcggcgacacactcggccgctgtgtacccggggcgcccggcgacaatgaggcacctgtggtgcagccttctgccacaagccttgcctacgtcatcttcacttccggctcgaccggcaagccgaagggtgtcatggtcgagcaccgtagtatcgtccgcttgatgaggcacagcaatgtctcgagtcgccttctgctacatccccgcatgacccacctgtcgaatctcgccttcgatgcgtcggtgtgggagattttcttgacgctgctcaacggtggaacattgatttgtattgactacctctcgtcactagactgtcgtgctcttggggtaagtatcctggaacaccaggttgacgcatcggtacttcctcctgctttgctcaaacaatgcctagcaaatgtccctgaggcacttgcgagcctgcaagtgctcttgtccgctggagatcgactcgacagtcgtgatgctatagagagttgcgcactcgtgcgcggaagtgtctacaatgggtatggtcccacggagaatggcatccagagcacaatctatgaagtcaaagcggacgctgagtttgtcaatggtgtgcctatcggccgcgctgtgagcaactcaggggcatatgtcatggacccgcagcagcaactggtgcctctcggggtgatgggcgagctcgtcgtcaccggcgacggcctggcccgtggttacaccgacccgtcactggatgcggaccgctttgtgcaggtctccgtcaacgggcagctcgtgagagcgtaccgaacaggcgatcgcgtgcgctgcaggccttgcgatggccagatcgagttctttggacgtatggaccggcaagtcaagatccgaggacatcgcatcgagctcgcagaggtagagcatgcggtgcttggcttggaagacgtgcaagacgctgccgttatcgcatttgacaatgtggacagcgaagagccagaaatggttgggtttgtcactattaccgaagacaatcctgtccgtgaggacgaaaccagcggtcaagtagaagactgggcgaaccacttcgagataagtacctacaccgatatcgcggcgatcgatcagggtagcattggaagtgactttgtaggttggacttctatgtacgacggaagcgagatcgacaaggcagagatgcaagaatggcttgccgataccatggcctctatgctcgacgggcaggcgccgggcaatgtgttagagataggtacaggcactggcatggtcctcttcaatctcggcgacggactgcagagctatgtcggcctcgaaccatcaagatcggcggccgcttttgtcaaccagacgattaagtcgctccccacccttgctggcaacgctgaagtacacattggcactgcgaccgacgtggcccgtctagatggcctccgccccgacttagtggtagtcaattcggtagtccagtacttcccatcaccagagtacctaatggaagtcgtggaggctcttgcacgtctgccgggcgtcgagcgaattttcttcggagacgtacgttcgtacgccatcaacagagatttcctggctgccagagctctacacgaacttggcgacagagcgactaagcacgagattcggcgaaagatgctagagatggaagaacgcgaagaggagctgctcgtcgacccagctttcttcaccatgttgaccagcagtctccctggcctgattcagcatgtcgagatcttgccgaagctgatgagagccactaatgagctcagcgcgtatcgatacactgctgtagtacacgtgtgccgtgccggtcaagagcctcgttccgtgcatacgatcgacgacgatgcctgggtgaatcttggagcttctcggttgagtcgccctaccctttcaagccttttgcaaacttccgagggcgcatcggccgtcgcagtaagcaatattccttacagcaagaccatcacagagcgagcgctcgttagtgcgctcgatgaggatgatatgcaagactcatcggactggctgctggccgtgcgcgagacaggcagatcttgttcctccttctccgcaacagaccttgtcgagcttgctcgagagacgggctggcgtgtggagctcagctgggcacgacagtactcacagaaaggcgcactcgatgctgtcttccacagacaccctgtttccgctgggagcgggcgtgtcatgttccagtttccagttgagaccgaagatcgaccgcacatctcacgcacgaaccgacctttacagcgattgcagaagaagcgaaccgagacacatgttcatgagcagttgcgggctttgcttccacgatacatggttcctacgcggattgtggcgcttgataagctgcccgtcaatgcaaacggcaaggttgatcgtcaacagctcgctaggacagcccaggttctcccagcgagcaaggcgccgtctgcatgcgtggccccacgcaacgaattggaaatgacactgtgtgaagagttctcgcaggttcttggcgtcgaggtcggcattactgacaatttcttccacctgggtggccactctctcatggcaacaaagcttgccgctcgtatcagccaccgccttcatacacgcatatccgtcaaacacatcttcgatcaccctttgataggcgatttgtctgtccacatagctgactctccggtgcctcttttgacaatcacacgtgcccagcacgctggagcagtggagcagtcattcgcacaagctagattgtggttccttgtccagctaggacttgaatctccttcgtacatcataccaattgtattgcgtttacacggttcactctcaaagactgccattgaaggagctctatcagccctgatggaacgtcatgaggtccttcgtacgacgttcgaggaccataagggtatcggcatgcaagtggtacaagaccatcgtcaccaagacttggttgtaattgacgttgcaggtcaggggtcactcgactacaagcagcacttatacatggagcacgtgaaacctttcgatctgacccgggatcctgggtggagggtagcgctgctgcgtctgggagatgacgaccacgtcctctccatcgtaatgcatcacatcatctccgatggctggtcgattgatatcctgctgcgtgagttgggtcagttctactcggccgcgctccgggggcaggacccgttgtcacagacaagtcctctgccgatccagtatcgtgacttcgctctctggcaaaagcaggatcatcaattagccgatcacgagaagcagctgcggtattgggaagagcaactggcggagagctctccagctgagctgctatgtgatcatgcacgtccgacgacgccctcaggtcaggcaggctcgattcccgtcaatgttcaaggctctctgtatcaggcgcttcgggcgttctgccgcgctcaccaggtcacctctttcgtagtcctgctcacggcgttccgcatagcacactatcgtctgacgggtgcggaggacgcaaccattggaactcccattgcaaatcgcaaccggccagagctcgagaacatgatcggtttcttcgtcaatacacaatgcatgcgcatcgtcattggcagtgacgacacatttgaagggctggtgcagcaagtacgctcgataactgcagctgcccacgagaaccaggacgttccattcgagcgcatcgtgtcagcactgcttcccggttctagagacacatcacgcaatcctctggtgcagttgttgttcgctgttcatgcctatcaagaggtcgaaaatttcgccatccccggtgtgcactccgagttggtgcaaggaacgacctttacaagatttgatgtcgagttccacctgcttgaagaccctgacaagctcagcggcaacgtgctcttcgcgaccgagctcttcgagcagaagactatgcaaggcatggtcgacgtgttccaggaagtgctcagccggggccttgagcagccccagatacctctggcgaccctcccgctcacgcacggactggaggagctcaggaccatgggtcttctcgacgtggagaagacagactaccctcgagagtcgagcgtggtggacgtgttccgtgagcaagcggctgcctgctccgaggcgattgcggtcaaagactcgtcggcgcagctcacctactcggagctcgatcgacagtcggacgagcttgccggctggctgcgccagcaacgtcttcctgcggagtcgttggttgcagtgctggcacccaggtcgtgccagaccattgtcgcgttcctgggcatcctcaaggcgaatctggcatacctgccgctagacgtcaacgtgcccgctactcgcctcgagtcgatactgtctgccgtcggcggccggaagctggtcttgcttggagctgacgtggccgaccctggccttcgcctggcggatgtggagctcgtgcggatcggcgacacactcggccgctgtgtacccggggcgcccggcgacaatgaggcacctgtggtgcagccttctgccacaagccttgcctacgtcatcttcacttccggctcgaccggcaagccgaagggtgtcatggtcgagcaccgcagtatactcagggttgtcacgtctcccccggcccgtgctctgctaccgtccacaatcatcatggcccacctgacaaacattgcattcgatgtatcgctatgggagatatgtacagctcttcttcacggtggtaccctgatctgtattcagtatcttgcctcgctcgatgtcagggggcttcagactacattctctcgcgaagctatcaacgtagctgtgtttcctcctgccttgctaaagacctgtcttgccaagattccatctgctctagcatcgctgagtgccatgttctcgtccggagatcgtctcgactcacgcgatgctagcgagggggccacacttgtgcggcaagggatacacaacgcgtatggtcccacggagaatggcatccagagcacaatctatgaagtcaaagcggacgctgagtttgtcaatggtgtgcctatcggccgcgctgtgagcaactcaggggcatatgtcatggacccgcagcagcaactggtgcctctcggggtgatgggcgagctcgtcgtcaccggcgacggcctggcccgtggttacaccgacccgtcactggatgcggaccgctttgtgcaggtctccgtcaacgggcagctcgtgagagcgtaccgaacaggcgatcgcgtgcgctgcaggccttgcgatggccagatcgagttctttggacgtatggaccggcaagtcaagatccgaggacatcgcatcgagctcgcagaggtagagcatgcgatattgtcccttgattatgtgatcgatgcagccgtccttctgagacagctgattgatcaagagccacaagtggtaggattcgtcattgtatccaccaaacgggcttattcccgacacaacagcggctacgcgtctgaagtttcggcattctgcatcaaagatcagatcgcatggcgcattcgacaacatctctgcaggatgctgccttcctatatggttccctatcaaattgcaattcttgatgaaatgcctatcaatgctaacggcaaggtggatagacagaatcttgcaagcagaactgtcaacgtccaaagaatcctcgccgctccatacatggccccgcgcaatgaagtcgagatttcgctttgcgaacagtatgctgccctgcttgaacacgacgttggcattcttgacgacttcttcgaacttggtggtcactctctcatggctactagactggcctcgcgtatcagctcccgattcagcgctccggtgtctgttcgtgatattttcgaccatccaagaatcatggaccttgctagcatcattcgtgctggagacattcaatggtcccggatactgccttctgcttatgaacgtccagtcgagcaatctttcgcacagaatcgcctgtggttcctgtacaagcttgacataggtacgacacagtataatttaccgctggcgatacaccttcgaggaccactagatatatcagcgctgtttatcgcattcaaggcattgactgaaagacatgaacttttgcgcacaacttttgatgaggatgacggaacatgcctgcagatgttattgcctgaatatcagcatgaagtaaggatcaccgacttgcagggatcacacaaaggtagcctcctggatattctcaacaacaatcagaagactcccttcgagctgagccgcgagcctggatggagggtagcgctgctgcgtctgggagatgacgaccacgtcctctccatcgtcatgcatcacatcatctccgacggttggtctgtggacgtgctgcgccacgagctaggtcagttctactcggccgcgctccgggggcaggacccgttgtcgcagataagtcctctgccgatccagtatcgtgacttcgctctctggcagagacaagacgagcaagttgcggagcatcagcgccagctggagcattggacagagcagttggcagacagttcacccgccgagttgttgagcgaccacccgaggccatcgattctttctggccaggcgggcgctattcccgtcaatgttcaaggctctctgtatcaggcgcttcgggcgttctgccgcgctcaccaggtcacctctttcgtagtcctgctcacggcgttccgcatagcacactatcgtctgacgggtgcggaggacgcaaccattggaactcccattgcaaatcgcaaccggccagagctcgagaacatgatcggtttcttcgtcaatacacaatgcatgcgcatcgtcattggcagtgacgacacatttgaagggctggtgcagcaagtacgctcgataactgcagctgcccacgagaaccaggacgttccattcgagcgcatcgtgtcagcactgcttcccggttctagagacacatcacgcaatcctctggttcagctcatgtttgctgtccactcgcaaagaaaccttggtcagatcagtctagaaggcctgcagggtgaattgctgggagtggcagcgactacgagattcgatgtagagttccatctcttccaagatgacgacaagctcagcggcaacgtgctcttcgcgaccgagctcttcgagcagaagactatgcaaggcatggtcgacgtgttccaggaagtgctcagccggggccttgagcagccccagatacctctggcgaccctcccgctcacgcacggactggaggagctcaggaccatgggtcttctcgacgtggagaagacagactaccctcgagagtcgagcgtggtggacgtgttccgtgagcaagcggctgcctgctccgaggcgattgcggtcaaagactcgtcggcgcagctcacctactcggagctcgatcgacagtcggacgagcttgccggctggctgcgccagcaacgtcttcctgcggagtcgttggttgcagtgctggcacccaggtcgtgccagaccattgtcgcgttcctgggcatcctcaaggcgaatctggcatacctgccgctagacgtcaacgtgcccgctactcgcctcgagtcgatactgtctgccgtcggcggccggaagctggtcttgcttggagctgacgtggccgaccctggccttcgcctggcggatgtggagctcgtgcggatcggcgacacactcggccgctgtgtacccggggcgcccggcgacaacgaggcacctgtggtgcagccttctgccacaagccttgcctacgtcatcttcacttccggctcgaccggcaagccgaagggtgtcatggtcgagcaccggggtgtagtgcgacttgtcaagcagagcaatgttgtctaccatctcccgtccacatctcgcgtggcccacctgtcgaatctcgcctttgatgcctcggtcctcgagatctatgcggcccttctgaacggtggtactgtttactgcattgactatctcactacccttgaccctcacgcgcttgagtctgttttcatcgatgctgatctcaacacggcagtccttcctcccgctctacttaaacaggtccttgcttcgagcccttctaccctccatgcccttgatttactcttcataggaggagatcgattggatgctcgtgacgccctgtacgctaatcgtctggttcgagggtcattatacaatgtctatggcccgacagagaacaccgttctgagcgtcgtttacctctttaatgatgacgatgcatgcattaatggcgtccctatcggccaagtcgtcagtaattccggggtatacgtcatggactcagaacagaaattagtacctcctggggtcatgggagaaatcgtcgtgacaggagacggtctcgcaagagggtatactgactcaaccttaaatactgatcgtttcgttcaaatcagtgtcaacggacgtgtactgcaagcataccgtacaggcgatcgtggtcggtaccgcccgacagacgctcgtcttgagttctttggccgtctagatcaacaaatcaagcttcgcgggcatcgtgtagagctcaaagaaatcgagcaagcgatgcttggccacaatgctgttgatgatgcaggagttgtcgctctggagatatctgagtgccaagagctagagatggttggctttgtgactctacgcaatcttggaaccatggaagcaactaacaatctcgcacacacaagctggaacccagtgactctcaaaacccctttagcatcacaaatagtggctgaggttcggggtagactccagcgaaatctgccactctatatggtacccgctacgattgtggtattacatactatgccagtcaatgccaacgggaagctcgaccgacaagcacttgtgaaagctgcaatgacgcttccaaaaactgctccactggtatggatggctccgcgcaatgaaggagagacatcgctatgtgaggagctaacagatatcttgggggtgaacgtcgggatcaccgataacttttttgaccttggggggcattccctcctggcaaccagagtagccgcgcgaatcagccgacgtcttgatgccctggtgaccgtcaaacaaatattcgaccatccagtcattggagatctcgcagctgcaattcaagggggttcagtacggcatttaccaataactgcaagcgaggtcgatggacctgttcagcagtccttcgcgcaaaatcgcttgtggttcctagagcagatgaatattggagctacttggtacatcgtaccgttagcagtgcgtctgtacggcacactgcgagttgaggctctgaatattgcgttgcgtacgattcagcaacgccacgaaacattacgaacgaccttcgaagaactaaatgggattgccgttcaacgttgtgattcaacctgccaaggccaattaagggtggtagatttagtcgggcaggggccagatcgctatagagagattctggatgtccagcaaactacaccattcgagctgagccaggagcctggatggagggtagcgctgcttcgtctgggagatgacgaccacgtcctctccatcgtcatgcatcacatcatctccgacggttggtctgtggacgtgctgctacgtgagataggtcagttctactcggccgcgctccgggggcaggacccgttgtcgcagataagtcctctgccgatccagtatcgtgacttcgctctctggcagagacaagacgagcaagttgcggagcatcagcgccagctggagcattggacagagcagttggcagacagttcacccgccgagttgttgagcgaccacccgaggccatcgattctttctggccaggcgggcgctattcccgtcaatgttcaaggctctctgtatcaggcgcttcgggcgttctgccgcgctcaccaggtcacctctttcgtagtcctgctcacggcgttccgcatagcacactatcgtctgacgggtgcggaggacgcaaccattggaactcccattgcaaatcgcaaccggccagagctcgagaacatgatcggtttcttcgtcaatacacaatgcatgcgcatcgtcattggcagtgacgacacatttgaagggctggtgcagcaagtacgctcgataactgcagctgcccacgagaaccaggacgttccattcgagcgcatcgtgtcagcactgcttcccggttctagagacacatcacgcaatcctctggttcagctcatgtttgctgtccactcgcaaagaaaccttggtcagatcagtctagaaggcctgcagggtgaattgctgggagtggcagcgactacgagattcgatgtagagttccatctcttccaagatgacgacaagctcagcggcaacgtgctcttcgcgaccgagctcttcgagcagaagactatgcaaggcatggtcgacgtgttccaggaagtgctcagccggggccttgagcagccccagatacctctggcgaccctcccgctcacgcacggactggaggagctcaggaccatgggtcttctcgacgtggagaagacagactaccctcgagagtcgagcgtggtggacgtgttccgtgagcaagcggctgcctgctccgaggcgattgcggtcaaagactcgtcggcgcagctcacctactcggagctcgatcgacagtcggacgagcttgccggctggctgcgccagcaacgtcttcctgcggagtcgttggttgcagtgctggcacccaggtcgtgccagaccattgtcgcgttcctgggcatcctcaaggcgaatctggcatacctgccgctagacgtcaacgtgcccgctactcgcctcgagtcgatactgtctgccgtcggcggccggaagctggtcttgcttggagctgacgtggccgaccctggccttcgcctggcggatgtggagctcgtgcggatcggcgacacactcggccgctgtgtacccggggcgcccggcgacaacgaggcacctgtggtgcagccttctgccacaagccttgcctacgtcatcttcacttccggctcgaccggcaagccgaagggtgtcatggtcgagcaccggggtgtagtgcgacttgtcaagcagagcaatgttgtctaccatctcccgtccacatctcgcgtggcccacctgtcgaatctcgcctttgatgcctcggcgtgggagatctatgcggcactgcttaatggcggtacactcatctgcattgactatttcacaactctagactgctctgctctcggcgccaaattcatcaaggagaagatcgtcgcgaccatgattccgccagcgcttctgaagcaatgtctggcgatcttcccgaccgctcttagtgaactggtcctgctgtttgctgccggagatcgattcagcagtggcgatgccgtcgaagtgcagcgccacaccaaaggcgctgtttgtaacgcgtacggaccgacagaaaacaccattcttagtacgatctacgaagtcaagcagaatgagaacttcccgaacggtgtgcctatcggccgcgctgtgagcaactcaggggcatatgtcatggacccgcagcagcaactggtgcctctcggggtgatgggcgagctcgtcgtcaccggcgacggcctggcccgtggttacaccgacccgtcactggatgcggaccgctttgtgcaggtctccgtcaacgggcagctcgtgagagcgtaccgaacaggcgatcgcgtgcgctgcaggccttgcgatggccagatcgagttctttggacgtatggaccggcaagtcaagatccgaggacatcgcatcgagctcgcagaggtagagcatgcggtgcttggcttggaagacgtgcaagacgctgccgttatcgcatttgacaatgtggacagcgaagagccagaaatggttgggtttgtcactattaccgaagacaatcctgtccgtgaggacgaaaccagcggtcaagtagaagactgggcgaaccacttcgagataagtacctacaccgatatcgcggcgatcgatcagggtagcattggaagtgactttgtaggttggacttctatgtacgacggaagcgagatcgacaaggcagagatgcaagaatggcttgccgataccatggcctctatgctcgacgggcaggcgccgggcaatgtgttagagataggtacaggcactggcatggtcctcttcaatctcggcgacggactgcagagctatgtcggcctcgaaccatcaagatcggcggccgcttttgtcaaccagacgattaagtcgctccccacccttgctggcaacgctgaagtacacattggcactgcgaccgacgtggcccgtctagatggcctccgccccgacttagtggtagtcaattcggtagtccagtacttcccatcaccagagtacctaatggaagtcgtggaggctcttgcacgtctgccgggcgtcgagcgaattttcttcggagacgtacgttcgtacgccatcaacagagatttcctggctgccagagctctacacgaacttggcgacagagcgactaagcacgagattcggcgaaagatgctagagatggaagaacgcgaagaggagctgctcgtcgacccagctttcttcaccatgttgaccagcagtctccctggcctgattcagcatgtcgagatcttgccgaagctgatgagagccactaatgagctcagcgcgtatcgatacactgctgtagtacacgtgtgccgtgccggtcaagagcctcgttccgtgcatacgatcgacgacgatgcctgggtgaatcttggagcttctcggttgagtcgccctaccctttcaagccttttgcaaacttccgagggcgcatcggccgtcgcagtaagcaatattccttacagcaagaccatcacagagcgagcgctcgttagtgcgctcgatgaggatgatatgcaagactcatcggactggctgctggccgtgcgcgagacaggcagatcttgttcctccttctccgcaacagaccttgtcgagcttgctcgagagacgggctggcgtgtggagctcagctgggcacgacagtactcacagaaaggcgcactcgatgctgtcttccacagacaccctgtttccgctgggagcgggcgtgtcatgttccagtttccagttgagaccgaagatcgaccgcacatctcacgcacgaaccgacctttacagcgattgcagaagaagcgaaccgagacacatgttcatgagcagttgcgggctttgcttccacgatacatggttcctacgcggattgtggcgcttgataagctgcccgtcaatgcaaacggcaaggttgatcgtcaacagctcgctaggacagcccaggttctcccagcgagcaaggcgccgtctgcatgcgtggccccacgcaacgaattggaaatgacactgtgtgaagagttctcgcaggttcttggcgtcgaggtcggcattactgacaatttcttccacctgggtggccactctctcatggcaacaaagttcgccgctcgtatcagccgccggctgaatgctatcgtttcggtcaagaatgtcttcgaccaccccgtacctatggatcttgcagcgacaatccaagaaggctcaaagcttcatactccaatccctcgcacggcttacagcggtcctgtcgaacagtctttcgcacaaggacgtctttggttccttgaccaattcaatcctagctcgattgggtatgtgatgcctttcgctgcgcgtcttcatggtcaactacaaatcgaagcgctcacagcagcattgttcgctttggaacagcgacatgagatcctgcgaacaacgttggacgcacacgatggtgtaggcatgcagatcgttcacgcggaacatccgcaacagttgagaatcattgatgtgtcagcaaaggcgtcgagcagttatgctcagacactgcgtgacgagcaggcgtcacctttcgacctaagcaaggaaccaggttggagagtctcgttgctgcagctcagtgagatagattatgttctttccattgtaatgcatcacaccatctatgacggttggtctctcgacgtactccggcgggagctaagtcagttttatgccgctgccatccgtggtcgagaacctctatcgacaatcgagccattgcctatccaataccgcgacttttctgtctggcaaaagcaggaagaccaagtcgcagagcatcgacgacagctccattattggatagagcagctagatggcagctctcctgctgagttcctaaacgataaaccacggcctacgttgctttctggcaaggcaggagttgtggaaattgctgtgaagggcactgtatatcaacgtctgctagagttctgcaggcttcatcaggtcacctcgttcatggtgctgcttgcggcattccgagcgacacactatcgtctgacaggcacagaggacgcgactgtcggaacacccatcgccaatcgcaatcgacctgagctggagaacatgattggattgttcgtgaatactcagtgtatacgcctcaagatcgaggacaatgatactctcgaggagctagtacagcacgttcgtgccacgatcacagcatcaatctcgaaccaggatgtaccctttgaacaggtagtgtctgcattgctaccaggatcacgcgacacctctaggaacccactagttcagctgacttttgcggtgcattctcagcgaaatttggctgacattcagctagaaaacgtggagaccaatgctatgccaatttgcccctcgacacgtttcgacgctgaattccacctcttccaagaggagaatatgctaagcggaagggtgctgttttcagacgatcttttcgagcagaagactatgcaaggcatggtcgacgtgttccaggaagtgctcagccggggccttgagcagccccagatacctctggcgaccctcccgctcacgcacggactggaggagctcaggaccatgggtcttctcgacgtggagaagacagactaccctcgagagtcgagcgtggtggacgtgttccgtgagcaagcggctgcctgctccgaggcgattgcggtcaaagactcgtcggcgcagctcacctactcggagctcgatcgacagtcggacgagcttgccggctggctgcgccagcaacgtcttcctgcggagtcgttggttgcagtgctggcacccaggtcgtgccagaccattgtcgcgttcctgggcatcctcaaggcgaatctggcatacctgccgctagacgtcaacgtgcccgctactcgcctcgagtcgatactgtctgccgtcggcggccggaagctggtcttgcttggagctgacgtggccgaccctggccttcgcctggcggatgtggagctcgtgcggatcggcgacacactcggccgctgtgtacccggggcgcccggcgacaacgaggcacctgtggtgcagccttctgccacaagccttgcctacgtcatcttcacttccggctcgaccggcaagccgaagggtgtcatggtcgagcaccggggtgtagtgcgacttgtcaagcagagcaatgttgtctaccatctcccgtccacatctcgcgtggcccacctgtcgaatctcgcctttgatgcctcggcgtgggagatctatgcggcactgcttaatggcggtacactcatctgcattgactatttcaccatcatagacgctcgcgcacttggcgttatctttgcgcaacaaagtatcaacgcaaccatgctgtcacctctactcctcaaacaatttttgtcagatgcaccattcgtgctgcgatctctgcatgccctttatctagggggggacagacttcagggtcgtgacgcaatccaggcttgtcgtgtaggttgcgcatttgtcatcaatgcctatggcccaacagagaattctgtcatcagtactacttacacacttgtgaagggaaatgcggacttcccgaacggtgtgcctatcggccgcgctgtgagcaactcaggggcatatgtcatggacccgcagcagcaactggtgcctctcggggtgatgggcgagctcgtcgtcaccggcgacggcctggcccgtggttacaccgacccgtcactggatgcggaccgctttgtgcaggtctccgtcaacgggcagctcgtgagagcgtaccgaacaggcgatcgcgtgcgctgcaggccttgcgatggccagatcgagttctttggacgtatggaccggcaagtcaagatccgaggacatcgcatcgagctcgcagaggtagagcatgcggtgcttggcttggaagacgtgcaagacgctgccgttctcatagctcaaacagccgaaaatgaagagctagttggcttcttcacgcttcgacaaacccaggctgtgcagtcaaatggtgccgctggtgttgtgccagagcacagcgactccgagctggcgcaatcctgctcttgcactcaaacggagcgtcgagtccgcaacagattgcaatcctgtcttcctcgctacatggttccgtcgcgaatggtccttttggatcgactgcctgtcaaccccaatggtaaagttgatcgacaagagctcacgaggcgcgctcaggatctcccaataagcgagtcatccccagtgcacgtcaaaccgcgtactgaactggaaaggtcgctgtgcgaggagttcgccgatgttataggtttggaagtcggcgttaccgataatttcttcgacctaggcgggcactctctcatggcgatgaaactcgcagctcgcatcagccgtcgttcgaatgcacatatatcagtcaaggacattttcgaccacccgctgattgcagatctcgcaatgaaaattcgggaaggctccgatctgcacactccaattccccacaggatgtacgttggacctatccagctatcattcgcacagggacgcttgtggttcctcgaccaattgaatttgggcgcatcgtggtacgtcatgccacttgctatgcgcctccaaggctcgctccagctcgacgcgttagagactgcactgtttgctatcgagcagcgacacgaaaccttacggatgacatttgcagaacaagacggagtagctgtacaagtagtgcatgcagcccactacaaacacatcaagatgatcgacaaaccacttagacagaagattgacgtcctgaagatgctggaagaagaacggacgactcccttcgagctgagccgcgagcctggatggagggtagcgctgctgcgtctgggagatgacgaccacgtcctctccatcgtcatgcatcacatcatctccgacggttggtctgtggacgtgctgcgccacgagctaggtcagttctactcggccgcgctccgggggcaggacccgttgtcgcagataagtcctctgccgatccagtatcgtgacttcgctctctggcagagacaagacgagcaagttgcggagcatcagcgccagctggagcattggacagagcagttggcagacagttcacccgccgagttgttgagcgaccacccgaggccatcgattctttctggccaggcgggcgctattcccgtcaatgttcaaggctctctgtatcaggcgcttcgggcgttctgccgcgctcaccaggtcacctctttcgtagtcctgctcacggcgttccgcatagcacactatcgtctgacgggtgcggaggacgcaaccattggaactcccattgcaaatcgcaaccggccagagctcgagaacatgatcggtttcttcgtcaatacacaatgcatgcgcatcgtcattggcagtgacgacacatttgaagggctggtgcagcaagtacgctcgataactgcagctgcccacgagaaccaggacgttccattcgagcgcatcgtgtcagcactgcttcccggttctagagacacatcacgcaatcctctggttcagctcatgtttgctgtccactcgcaaagaaaccttggtcagatcagtctagaaggcctgcagggtgaattgctgggagtggcagcgactacgagattcgatgtagagttccatctcttccaagatgacgacaagctcagcggcaacgtgctcttcgcgaccgagctcttcgagcagaagactatgcaaggcatggtcgacgtgttccaggaagtgctcagccggggccttgagcagccccagatacctctggcgaccctcccgctcacgcacggactggaggagctcaggaccatgggtcttctcgacgtggagaagacagactaccctcgagagtcgagcgtggtggacgtgttccgtgagcaagcggctgcctgctccgaggcgattgcggtcaaagactcgtcggcgcagctcacctactcggagctcgatcgacagtcggacgagcttgccggctggctgcgccagcaacgtcttcctgcggagtcgttggttgcagtgctggcacccaggtcgtgccagaccattgtcgcgttcctgggcatcctcaaggcgaatctggcatacctgccgctagacgtcaacgtgcccgctactcgcctcgagtcgatactgtctgccgtcggcggccggaagctggtcttgcttggagctgacgtggccgaccctggccttcgcctggcggatgtggagctcgtgcggatcggcgacacactcggccgctgtgtacccggggcgcccggcgacaacgaggcacctgtggtgcagccttctgccacaagccttgcctacgtcatcttcacttccggctcgaccggcaagccgaagggtgtcatggtcgagcaccggggtgtagtgcgacttgtcaagcagagcaatgttgtctaccatctcccgtccacatctcgcgtggcccacctgtcgaatctcgcctttgatgcctcggcgtgggagatctatgcggcactgcttaatggcggtacactcatctgcattgactatttcacaactctagactgctctgctctcggcgccaaattcatcaaggagaagatcgtcgcgaccatgattccgccagcgcttctgaagcaatgtctggcgatcttcccgaccgctcttagtgaactggtcctgctgtttgctgccggagatcgattcagcagtggcgatgccgtcgaagtgcagcgccacaccaaaggcgctgtttgtaacgcgtacggaccgacagaaaacaccattcttagtacgatctacgaagtcaagcagaatgagaacttcccgaacggtgtgcctatcggccgcgctgtgagcaactcaggggcatatgtcatggacccgcagcagcaactggtgcctctcggggtgatgggcgagctcgtcgtcaccggcgacggcctggcccgtggttacaccgacccgtcactggatgcggaccgctttgtgcaggtctccgtcaacgggcagctcgtgagagcgtaccgaacaggcgatcgcgtgcgctgcaggccttgcgatggccagatcgagttctttggacgtatggaccggcaagtcaagatccgaggacatcgcatcgagctcgcagaggtagagcatgcggtgcttggcttggaagacgtgcaagacgctgccgttatcgcatttgacaatgtggacagcgaagagccagaaatggttgggtttgtcactattaccgaagacaatcctgtccgtgaggacgaaaccagcggtcaagtagaagactgggcgaaccacttcgagataagtacctacaccgatatcgcggcgatcgatcagggtagcattggaagtgactttgtaggttggacttctatgtacgacggaagcgagatcgacaaggcagagatgcaagaatggcttgccgataccatggcctctatgctcgacgggcaggcgccgggcaatgtgttagagataggtacaggcactggcatggtcctcttcaatctcggcgacggactgcagagctatgtcggcctcgaaccatcaagatcggcggccgcttttgtcaaccagacgattaagtcgctccccacccttgctggcaacgctgaagtacacattggcactgcgaccgacgtggcccgtctagatggcctccgccccgacttagtggtagtcaattcggtagtccagtacttcccatcaccagagtacctaatggaagtcgtggaggctcttgcacgtctgccgggcgtcgagcgaattttcttcggagacgtacgttcgtacgccatcaacagagatttcctggctgccagagctctacacgaacttggcgacagagcgactaagcacgagattcggcgaaagatgctagagatggaagaacgcgaagaggagctgctcgtcgacccagctttcttcaccatgttgaccagcagtctccctggcctgattcagcatgtcgagatcttgccgaagctgatgagagccactaatgagctcagcgcgtatcgatacactgctgtagtacacgtgtgccgtgccggtcaagagcctcgttccgtgcatacgatcgacgacgatgcctgggtgaatcttggagcttctcggttgagtcgccctaccctttcaagccttttgcaaacttccgagggcgcatcggccgtcgcagtaagcaatattccttacagcaagaccatcacagagcgagcgctcgttagtgcgctcgatgaggatgatatgcaagactcatcggactggctgctggccgtgcgcgagacaggcagatcttgttcctccttctccgcaacagaccttgtcgagcttgctcgagagacgggctggcgtgtggagctcagctgggcacgacagtactcacagaaaggcgcactcgatgctgtcttccacagacaccctgtttccgctgggagcgggcgtgtcatgttccagtttccagttgagaccgaagatcgaccgcacatctcacgcacgaaccgacctttacagcgattgcagaagaagcgaaccgagacacatgttcatgagcagttgcgggctttgcttccacgatacatggttcctacgcggattgtggcgcttgataagctgcccgtcaatgcaaacggcaaggttgatcgtcaacagctcgctaggacagcccaggttctcccagcgagcaaggcgccgtctgcatgcgtggccccacgcaacgaattggaaatgacactgtgtgaagagttctcgcaggttcttggcgtcgaggtcggcattactgacaatttcttccacctgggtggccactctctcatggcaacaaagcttgccgctcgtatcagccgtcaactaaatatccaagtctcagtccgagacatctttgactatcccgttatagtcgacctcacagacagattgagactccatcatacgcgtatccttactcatgatcatggacaacatggacagccagacctcaagccattcaccttgctaccaaccaacaatcctcaagaattcctacagcatcacattttgccacaacttgttcccgatcatgcgaagatcctcgatgtgtatcccgttacaagaatacagagaaggtttcttcatcatccgaagcgcggcctccctcgttttccctccatggtcttctttgacttccctcctggttcagacccacacaagctaagattagcttgtatggcattagtccagcgtttcgacattcttcgcacaatcttcctttctgtttcgggtcaattcttccaagtggtcctggatggatatgggattgtcataccggtcatcgaggttgacgaagagctagacgacgccacccgtaaattacacgattccgatattcagcagcccttacggttgggaaaaccgttaatacgcattgctgtcttgaaaaggcagcactccagagtacgagcagtcttgcgcttgtcgcatgctctctatgatggtttgagctttgagcatatcatccaatctcttcatgccctttatctcgatatcaccctttcggccccaccgaagtttggactctacgtacaacatatgatacaaagtcgcgcagaaggttatgctttctggcggtctgtcttgaagggctcgtcgatgacaattctcgagcgttctagcacccttcaatcgcggcagccgcatcttggacgttttctctctgcggagaaaattattaaggctcctttacacgccaacaagtctggaatcacacaggcaacagtgttcgcggccgcaaacgcactcatgcttgcgaatcttactggtactaatgacgttgtgtttgcccgcattgtctctggacgtcaatctttgcctaagaactttcagcacgttgtgggaccttgcacgaacgatgtgcccgttcgcgtacgcatggagcctggcgtgggaccaaaagctttactcagacaggtgcaagaccagtatgttcatagcttccctttcgaaacactaggattcgacgagatcaaggagaactgtacggactggccagaaagaatcacgaattttgggtgttctacaacttaccagaactttgacatttttcccaaaagtcagattgaccaccagcagattcaaatggctagcttggcaagcgagtatcagaatcgagaaacctgggacgaagcgccgctatacgacctcaatgtcacaggagtacctcagcctgacggacgtcatatcaagatatacgtgggtgtagacgggcagctttgcgatgaaagcacgcttgattgcattctctcggatatttgtgagggtgtggtctcgctcacagacgctttgcaagaacttcccgctgctagcattactgagtagaatcccaagagagcaacaccctatcatgatagcgacagcacgttttcagttcgtcagagcttgactgaaatgcttttcgtctactacatctagcgtgtcataccagctagtagctacaacggagcaacgattggctgatgagccaggacctgaaaagaagaagaagatggaaatatagccttggaatctataataaag

SEQ ID NO: 6 - protein, 11659 aa, Aureobasidium pullulans strain BP-1938
MSRMPQGAARRNDCVSEHQGTTDLEDIVRFWERHLDGVNASAFPALSSSLVVPKPKLQTEHRISLGTAVSDQWSDAVICRAALAVILARYTHATEALYGIVVEQPSVSNAQKRSADDASSIVVPIRVQCASGQFGNDILAAIATHDASCRSLSAIGLDGIRCLDDAKTVARGLQTVLTVTSRKSVDASSPNILDLENIASSHGRALMIECQMSTTSACLRAQYDAGILRNEQVVRLLKQLALSIQHFRGNAANDLLRDFCFISPGEEMEIAYWNRRSIRTNEVCIHDVIFKRATYMPTDTAVSAWDGEWTYADLDVVSSCLADYVRSLDLRSGQAIPLCFEKSRNTIAAMVAVLKAGHPFCLIDPSTPSARITQMCEQMSATVAFASRALCSIMQAGVSRCIAVDDDLFQSLSSVIGCPQMSMTRPQDLAYVIFTSGSTGIPKGSMIEHRGFASCALEFGPQLLIDRNTRALQFASHAFGACLLEVLVTLMLGGCVCVPSENDRLNNLSGFIEQSGVNWTLFTPSFIGALTPETIRGVHTVVLGGEPMTPFIRDVWASKVQLLSIYGQSESSTVCSVVKIKPDTTDLSSLGHAIGARFWIVDAENPSRLAPIGCIGELMVESPGIAREYLSAQEAQMSPFITKTPAWYPMKQRCSPVKFYMTGDLACYGRDGTVMNLGRKDSQVKIRGQRVELGDVETNLRSVLPKHIIPVVEAIDSIHASGSKFLVAILIGANHGMKNEFDTEPRREVSILDETAVIRIRKSMQDLVPSYCIPTQYICMERLLTTTTGKADRKRLRAICVDLLKPSRRAMVPESSDGPTLKLTAGQVLDEAWHRYLRFDSVLDGSKSKFFDLNGDSITAIKIANAARKHGVMLKVADILANPTLADLRAQFQIDFTPQNSILRTSYRGPIQQSFAQNRLWFLDQLNVGASWYIVPVAVRLQGTVHVDALVTALCALEQRHETLRTTFEESDGEGIQRIQPSGLEQLRLIDVDCVDSRDYQRVLEEEQTTPFELSREPGWRVALLRLGDDDHVLSIVMHHIISDGWSVDVLRHELGQFYSAALRGQDPLSQISPLPIQYRDFALWQRQDEQVAEHQRQLEHWTEQLADSSPAELLSDHPRPSILSGQAGAIPVNVQGSLYQALRAFCRAHQVTSFVVLLTAFRIAHYRLTGAEDATIGTPIANRNRPELENMIGFFVNTQCMRIVIGSDDTFEGLVQQVRSITAAAHENQDVPFERIVSALLPGSRDTSRNPLVQLMFAVHSQRNLGQISLEGLQGELLGVASPTRFDVEFHLFQEENMLSGRVLFSDDLFEQKTMQGMVDVFQEVLSRGLEQPQIPLATLPLTHGLEELRTMGLLDVEKTDYPRESSVVDVFREQAAACSEAIAVKDSSAQLTYSELDRQSDELAGWLRQQRLPAESLVAVLAPRSCQTIVAFLGILKANLAYLPLDVNVPATRLESILSAVGGRKLVLLGADVADPGLRLADVELVRIGDTLGRCVPGAPGDNEAPVVQPSATSLAYVIFTSGSTGKPKGVMVEHRGVVRLVKQSNVVYHLPSTSRVAHLSNLAFDASAWEIYAALLNGGTLICIDYFTTLDCSALGAKFIKEKIVATMIPPALLKQCLAIFPTALSELVLLFAAGDRFSSGDAVEVQRHTKGAVCNAYGPTENTILSTIYEVKQNENFPNGVPIGRAVSNSGAYVMDPQQQLVPLGVMGELVVTGDGLARGYTDPSLDADRFVQVSVNGQLVRAYRTGDRVRCRPCDGQIEFFGRMDRQVKIRGHRIELAEVEHAVLGLEDVQDAAVIAFDNVDSEEPEMVGFVTITEDNPVREDETSGQVEDWANHFEISTYTDIAAIDQGSIGSDFVGWTSMYDGSEIDKAEMQEWLADTMASMLDGQAPGNVLEIGTGTGMVLFNLGDGLQSYVGLEPSRSAAAFVNQTIKSLPTLAGNAEVHIGTATDVARLDGLRPDLVVVNSVVQYFPSPEYLMEVVEALARLPGVERIFFGDVRSYAINRDFLAARALHELGDRATKHEIRRKMLEMEEREEELLVDPAFFTMLTSSLPGLIQHVEILPKLMRATNELSAYRYTAVVHVCRAGQEPRSVHTIDDDAWVNLGASRLSRPTLSSLLQTSEGASAVAVSNIPYSKTITERALVSALDEDDMQDSSDWLLAVRETGRSCSSFSATDLVELARETGWRVELSWARQYSQKGALDAVFHRHPVSAGSGRVMFQFPVETEDRPHISRTNRPLQRLQKKRTETHVHEQLRALLPRYMVPTRIVALDKLPVNANGKVDRQQLARTAQVLPASKAPSACVAPRNELEMTLCEEFSQVLGVEVGITDNFFHLGGHSLMATKFAARISRRLNAIVSVKNVFDHPVPMDLAATIQEGSKLHTPIPRTAYSGPVEQSFAQGRLWFLDQFNPSSIGYVMPFAARLHGQLQIEALTAALFALEQRHEILRTTLDAHDGVGMQIVHAEHPQQLRIIDVSAKASSSYAQTLRDEQASPFDLSKEPGWRVSLLQLSEIDYVLSIVMHHTIYDGWSLDVLRRELSQFYAAAIRGREPLSTIEPLPIQYRDFSVWQKQEDQVAEHRRQLHYWIEQLDGSSPAEFLNDKPRPTLLSGKAGVVEIAVKGTVYQRLLEFCRLHQVTSFMVLLAAFRATHYRLTGTEDATVGTPIANRNRPELENMIGLFVNTQCIRLKIEDNDTLEELVQHVRATITASISNQDVPFEQVVSALLPGSRDTSRNPLVQLTFAVHSQRNLADIQLENVETNAMPICPSTRFDAEFHLFQEENMLSGRVLFSDDLFEQKTMQGMVDVFQEVLSRGLEQPQIPLATLPLTHGLEELRTMGLLDVEKTDYPRESSVVDVFREQAAACSEAIAVKDSSAQLTYSELDRQSDELAGWLRQQRLPAESLVAVLAPRSCQTIVAFLGILKANLAYLPLDVNVPATRLESILSAVGGRKLVLLGADVADPGLRLADVELVRIGDTLGRCVPGAPGDNEAPVVQPSATSLAYVIFTSGSTGKPKGVMVEHRSIVRLMRHSNVSSRLLLHPRMTHLSNLAFDASVWEIFLTLLNGGTLICIDYLSSLDCRALGVSILEHQVDASVLPPALLKQCLANVPEALASLQVLLSAGDRLDSRDAIESCALVRGSVYNGYGPTENGIQSTIYEVKADAEFVNGVPIGRAVSNSGAYVMDPQQQLVPLGVMGELVVTGDGLARGYTDPSLDADRFVQVSVNGQLVRAYRTGDRVRCRPCDGQIEFFGRMDRQVKIRGHRIELAEVEHAVLGLEDVQDAAVLIAQTAENEELVGFFTLRQTQAVQSNGAAGVVPEHSDSELAQSCSCTQTERRVRNRLQSCLPRYMVPSRMVLLDRLPVNPNGKVDRQELTRRAQDLPISESSPVHVKPRTELERSLCEEFADVIGLEVGVTDNFFDLGGHSLMAMKLAARISRRSNAHISVKDIFDHPLIADLAMKIREGSDLHTPIPHRMYVGPIQLSFAQGRLWFLDQLNLGASWYVMPLAMRLQGSLQLDALETALFAIEQRHETLRMTFAEQDGVAVQVVHAAHYKHIKMIDKPLRQKIDVLKMLEEERTTPFELSREPGWRVALLRLGDDDHVLSIVMHHIISDGWSVDVLRHELGQFYSAALRGQDPLSQISPLPIQYRDFALWQRQDEQVAEHQRQLEHWTEQLADSSPAELLSDHPRPSILSGQAGAIPVNVQGSLYQALRAFCRAHQVTSFVVLLTAFRIAHYRLTGAEDATIGTPIANRNRPELENMIGFFVNTQCMRIVIGSDDTFEGLVQQVRSITAAAHENQDVPFERIVSALLPGSRDTSRNPLVQLMFAVHSQRNLGQISLEGLQGELLGVAATTRFDVEFHLFQDDDKLSGNVLFATELFEQKTMQGMVDVFQEVLSRGLEQPQIPLATLPLTHGLEELRTMGLLDVEKTDYPRESSVVDVFREQAAACSEAIAVKDSSAQLTYSELDRQSDELAGWLRQQRLPAESLVAVLAPRSCQTIVAFLGILKANLAYLPLDVNVPATRLESILSAVGGRKLVLLGADVADPGLRLADVELVRIGDTLGRCVPGAPGDNEAPVVQPSATSLAYVIFTSGSTGKPKGVMVEHRSIVRLMRHSNVSSRLLLHPRMTHLSNLAFDASVWEIFLTLLNGGTLICIDYLSSLDCRALGVSILEHQVDASVLPPALLKQCLANVPEALASLQVLLSAGDRLDSRDAIESCALVRGSVYNGYGPTENGIQSTIYEVKADAEFVNGVPIGRAVSNSGAYVMDPQQQLVPLGVMGELVVTGDGLARGYTDPSLDADRFVQVSVNGQLVRAYRTGDRVRCRPCDGQIEFFGRMDRQVKIRGHRIELAEVEHAVLGLEDVQDAAVIAFDNVDSEEPEMVGFVTITEDNPVREDETSGQVEDWANHFEISTYTDIAAIDQGSIGSDFVGWTSMYDGSEIDKAEMQEWLADTMASMLDGQAPGNVLEIGTGTGMVLFNLGDGLQSYVGLEPSRSAAAFVNQTIKSLPTLAGNAEVHIGTATDVARLDGLRPDLVVVNSVVQYFPSPEYLMEVVEALARLPGVERIFFGDVRSYAINRDFLAARALHELGDRATKHEIRRKMLEMEEREEELLVDPAFFTMLTSSLPGLIQHVEILPKLMRATNELSAYRYTAVVHVCRAGQEPRSVHTIDDDAWVNLGASRLSRPTLSSLLQTSEGASAVAVSNIPYSKTITERALVSALDEDDMQDSSDWLLAVRETGRSCSSFSATDLVELARETGWRVELSWARQYSQKGALDAVFHRHPVSAGSGRVMFQFPVETEDRPHISRTNRPLQRLQKKRTETHVHEQLRALLPRYMVPTRIVALDKLPVNANGKVDRQQLARTAQVLPASKAPSACVAPRNELEMTLCEEFSQVLGVEVGITDNFFHLGGHSLMATKLAARISHRLHTRISVKHIFDHPLIGDLSVHIADSPVPLLTITRAQHAGAVEQSFAQARLWFLVQLGLESPSYIIPIVLRLHGSLSKTAIEGALSALMERHEVLRTTFEDHKGIGMQVVQDHRHQDLVVIDVAGQGSLDYKQHLYMEHVKPFDLTRDPGWRVALLRLGDDDHVLSIVMHHIISDGWSIDILLRELGQFYSAALRGQDPLSQTSPLPIQYRDFALWQKQDHQLADHEKQLRYWEEQLAESSPAELLCDHARPTTPSGQAGSIPVNVQGSLYQALRAFCRAHQVTSFVVLLTAFRIAHYRLTGAEDATIGTPIANRNRPELENMIGFFVNTQCMRIVIGSDDTFEGLVQQVRSITAAAHENQDVPFERIVSALLPGSRDTSRNPLVQLLFAVHAYQEVENFAIPGVHSELVQGTTFTRFDVEFHLLEDPDKLSGNVLFATELFEQKTMQGMVDVFQEVLSRGLEQPQIPLATLPLTHGLEELRTMGLLDVEKTDYPRESSVVDVFREQAAACSEAIAVKDSSAQLTYSELDRQSDELAGWLRQQRLPAESLVAVLAPRSCQTIVAFLGILKANLAYLPLDVNVPATRLESILSAVGGRKLVLLGADVADPGLRLADVELVRIGDTLGRCVPGAPGDNEAPVVQPSATSLAYVIFTSGSTGKPKGVMVEHRSILRVVTSPPARALLPSTIIMAHLTNIAFDVSLWEICTALLHGGTLICIQYLASLDVRGLQTTFSREAINVAVFPPALLKTCLAKIPSALASLSAMFSSGDRLDSRDASEGATLVRQGIHNAYGPTENGIQSTIYEVKADAEFVNGVPIGRAVSNSGAYVMDPQQQLVPLGVMGELVVTGDGLARGYTDPSLDADRFVQVSVNGQLVRAYRTGDRVRCRPCDGQIEFFGRMDRQVKIRGHRIELAEVEHAILSLDYVIDAAVLLRQLIDQEPQVVGFVIVSTKRAYSRHNSGYASEVSAFCIKDQIAWRIRQHLCRMLPSYMVPYQIAILDEMPINANGKVDRQNLASRTVNVQRILAAPYMAPRNEVEISLCEQYAALLEHDVGILDDFFELGGHSLMATRLASRISSRFSAPVSVRDIFDHPRIMDLASIIRAGDIQWSRILPSAYERPVEQSFAQNRLWFLYKLDIGTTQYNLPLAIHLRGPLDISALFIAFKALTERHELLRTTFDEDDGTCLQMLLPEYQHEVRITDLQGSHKGSLLDILNNNQKTPFELSREPGWRVALLRLGDDDHVLSIVMHHIISDGWSVDVLRHELGQFYSAALRGQDPLSQISPLPIQYRDFALWQRQDEQVAEHQRQLEHWTEQLADSSPAELLSDHPRPSILSGQAGAIPVNVQGSLYQALRAFCRAHQVTSFVVLLTAFRIAHYRLTGAEDATIGTPIANRNRPELENMIGFFVNTQCMRIVIGSDDTFEGLVQQVRSITAAAHENQDVPFERIVSALLPGSRDTSRNPLVQLMFAVHSQRNLGQISLEGLQGELLGVAATTRFDVEFHLFQDDDKLSGNVLFATELFEQKTMQGMVDVFQEVLSRGLEQPQIPLATLPLTHGLEELRTMGLLDVEKTDYPRESSVVDVFREQAAACSEAIAVKDSSAQLTYSELDRQSDELAGWLRQQRLPAESLVAVLAPRSCQTIVAFLGILKANLAYLPLDVNVPATRLESILSAVGGRKLVLLGADVADPGLRLADVELVRIGDTLGRCVPGAPGDNEAPVVQPSATSLAYVIFTSGSTGKPKGVMVEHRGVVRLVKQSNVVYHLPSTSRVAHLSNLAFDASVLEIYAALLNGGTVYCIDYLTTLDPHALESVFIDADLNTAVLPPALLKQVLASSPSTLHALDLLFIGGDRLDARDALYANRLVRGSLYNVYGPTENTVLSVVYLFNDDDACINGVPIGQVVSNSGVYVMDSEQKLVPPGVMGEIVVTGDGLARGYTDSTLNTDRFVQISVNGRVLQAYRTGDRGRYRPTDARLEFFGRLDQQIKLRGHRVELKEIEQAMLGHNAVDDAGVVALEISECQELEMVGFVTLRNLGTMEATNNLAHTSWNPVTLKTPLASQIVAEVRGRLQRNLPLYMVPATIVVLHTMPVNANGKLDRQALVKAAMTLPKTAPLVWMAPRNEGETSLCEELTDILGVNVGITDNFFDLGGHSLLATRVAARISRRLDALVTVKQIFDHPVIGDLAAAIQGGSVRHLPITASEVDGPVQQSFAQNRLWFLEQMNIGATWYIVPLAVRLYGTLRVEALNIALRTIQQRHETLRTTFEELNGIAVQRCDSTCQGQLRVVDLVGQGPDRYREILDVQQTTPFELSQEPGWRVALLRLGDDDHVLSIVMHHIISDGWSVDVLLREIGQFYSAALRGQDPLSQISPLPIQYRDFALWQRQDEQVAEHQRQLEHWTEQLADSSPAELLSDHPRPSILSGQAGAIPVNVQGSLYQALRAFCRAHQVTSFVVLLTAFRIAHYRLTGAEDATIGTPIANRNRPELENMIGFFVNTQCMRIVIGSDDTFEGLVQQVRSITAAAHENQDVPFERIVSALLPGSRDTSRNPLVQLMFAVHSQRNLGQISLEGLQGELLGVAATTRFDVEFHLFQDDDKLSGNVLFATELFEQKTMQGMVDVFQEVLSRGLEQPQIPLATLPLTHGLEELRTMGLLDVEKTDYPRESSVVDVFREQAAACSEAIAVKDSSAQLTYSELDRQSDELAGWLRQQRLPAESLVAVLAPRSCQTIVAFLGILKANLAYLPLDVNVPATRLESILSAVGGRKLVLLGADVADPGLRLADVELVRIGDTLGRCVPGAPGDNEAPVVQPSATSLAYVIFTSGSTGKPKGVMVEHRGVVRLVKQSNVVYHLPSTSRVAHLSNLAFDASAWEIYAALLNGGTLICIDYFTTLDCSALGAKFIKEKIVATMIPPALLKQCLAIFPTALSELVLLFAAGDRFSSGDAVEVQRHTKGAVCNAYGPTENTILSTIYEVKQNENFPNGVPIGRAVSNSGAYVMDPQQQLVPLGVMGELVVTGDGLARGYTDPSLDADRFVQVSVNGQLVRAYRTGDRVRCRPCDGQIEFFGRMDRQVKIRGHRIELAEVEHAVLGLEDVQDAAVIAFDNVDSEEPEMVGFVTITEDNPVREDETSGQVEDWANHFEISTYTDIAAIDQGSIGSDFVGWTSMYDGSEIDKAEMQEWLADTMASMLDGQAPGNVLEIGTGTGMVLFNLGDGLQSYVGLEPSRSAAAFVNQTIKSLPTLAGNAEVHIGTATDVARLDGLRPDLVVVNSVVQYFPSPEYLMEVVEALARLPGVERIFFGDVRSYAINRDFLAARALHELGDRATKHEIRRKMLEMEEREEELLVDPAFFTMLTSSLPGLIQHVEILPKLMRATNELSAYRYTAVVHVCRAGQEPRSVHTIDDDAWVNLGASRLSRPTLSSLLQTSEGASAVAVSNIPYSKTITERALVSALDEDDMQDSSDWLLAVRETGRSCSSFSATDLVELARETGWRVELSWARQYSQKGALDAVFHRHPVSAGSGRVMFQFPVETEDRPHISRTNRPLQRLQKKRTETHVHEQLRALLPRYMVPTRIVALDKLPVNANGKVDRQQLARTAQVLPASKAPSACVAPRNELEMTLCEEFSQVLGVEVGITDNFFHLGGHSLMATKFAARISRRLNAIVSVKNVFDHPVPMDLAATIQEGSKLHTPIPRTAYSGPVEQSFAQGRLWFLDQFNPSSIGYVMPFAARLHGQLQIEALTAALFALEQRHEILRTTLDAHDGVGMQIVHAEHPQQLRIIDVSAKASSSYAQTLRDEQASPFDLSKEPGWRVSLLQLSEIDYVLSIVMHHTIYDGWSLDVLRRELSQFYAAAIRGREPLSTIEPLPIQYRDFSVWQKQEDQVAEHRRQLHYWIEQLDGSSPAEFLNDKPRPTLLSGKAGVVEIAVKGTVYQRLLEFCRLHQVTSFMVLLAAFRATHYRLTGTEDATVGTPIANRNRPELENMIGLFVNTQCIRLKIEDNDTLEELVQHVRATITASISNQDVPFEQVVSALLPGSRDTSRNPLVQLTFAVHSQRNLADIQLENVETNAMPICPSTRFDAEFHLFQEENMLSGRVLFSDDLFEQKTMQGMVDVFQEVLSRGLEQPQIPLATLPLTHGLEELRTMGLLDVEKTDYPRESSVVDVFREQAAACSEAIAVKDSSAQLTYSELDRQSDELAGWLRQQRLPAESLVAVLAPRSCQTIVAFLGILKANLAYLPLDVNVPATRLESILSAVGGRKLVLLGADVADPGLRLADVELVRIGDTLGRCVPGAPGDNEAPVVQPSATSLAYVIFTSGSTGKPKGVMVEHRGVVRLVKQSNVVYHLPSTSRVAHLSNLAFDASAWEIYAALLNGGTLICIDYFTIIDARALGVIFAQQSINATMLSPLLLKQFLSDAPFVLRSLHALYLGGDRLQGRDAIQACRVGCAFVINAYGPTENSVISTTYTLVKGNADFPNGVPIGRAVSNSGAYVMDPQQQLVPLGVMGELVVTGDGLARGYTDPSLDADRFVQVSVNGQLVRAYRTGDRVRCRPCDGQIEFFGRMDRQVKIRGHRIELAEVEHAVLGLEDVQDAAVLIAQTAENEELVGFFTLRQTQAVQSNGAAGVVPEHSDSELAQSCSCTQTERRVRNRLQSCLPRYMVPSRMVLLDRLPVNPNGKVDRQELTRRAQDLPISESSPVHVKPRTELERSLCEEFADVIGLEVGVTDNFFDLGGHSLMAMKLAARISRRSNAHISVKDIFDHPLIADLAMKIREGSDLHTPIPHRMYVGPIQLSFAQGRLWFLDQLNLGASWYVMPLAMRLQGSLQLDALETALFAIEQRHETLRMTFAEQDGVAVQVVHAAHYKHIKMIDKPLRQKIDVLKMLEEERTTPFELSREPGWRVALLRLGDDDHVLSIVMHHIISDGWSVDVLRHELGQFYSAALRGQDPLSQISPLPIQYRDFALWQRQDEQVAEHQRQLEHWTEQLADSSPAELLSDHPRPSILSGQAGAIPVNVQGSLYQALRAFCRAHQVTSFVVLLTAFRIAHYRLTGAEDATIGTPIANRNRPELENMIGFFVNTQCMRIVIGSDDTFEGLVQQVRSITAAAHENQDVPFERIVSALLPGSRDTSRNPLVQLMFAVHSQRNLGQISLEGLQGELLGVAATTRFDVEFHLFQDDDKLSGNVLFATELFEQKTMQGMVDVFQEVLSRGLEQPQIPLATLPLTHGLEELRTMGLLDVEKTDYPRESSVVDVFREQAAACSEAIAVKDSSAQLTYSELDRQSDELAGWLRQQRLPAESLVAVLAPRSCQTIVAFLGILKANLAYLPLDVNVPATRLESILSAVGGRKLVLLGADVADPGLRLADVELVRIGDTLGRCVPGAPGDNEAPVVQPSATSLAYVIFTSGSTGKPKGVMVEHRGVVRLVKQSNVVYHLPSTSRVAHLSNLAFDASAWEIYAALLNGGTLICIDYFTTLDCSALGAKFIKEKIVATMIPPALLKQCLAIFPTALSELVLLFAAGDRFSSGDAVEVQRHTKGAVCNAYGPTENTILSTIYEVKQNENFPNGVPIGRAVSNSGAYVMDPQQQLVPLGVMGELVVTGDGLARGYTDPSLDADRFVQVSVNGQLVRAYRTGDRVRCRPCDGQIEFFGRMDRQVKIRGHRIELAEVEHAVLGLEDVQDAAVIAFDNVDSEEPEMVGFVTITEDNPVREDETSGQVEDWANHFEISTYTDIAAIDQGSIGSDFVGWTSMYDGSEIDKAEMQEWLADTMASMLDGQAPGNVLEIGTGTGMVLFNLGDGLQSYVGLEPSRSAAAFVNQTIKSLPTLAGNAEVHIGTATDVARLDGLRPDLVVVNSVVQYFPSPEYLMEVVEALARLPGVERIFFGDVRSYAINRDFLAARALHELGDRATKHEIRRKMLEMEEREEELLVDPAFFTMLTSSLPGLIQHVEILPKLMRATNELSAYRYTAVVHVCRAGQEPRSVHTIDDDAWVNLGASRLSRPTLSSLLQTSEGASAVAVSNIPYSKTITERALVSALDEDDMQDSSDWLLAVRETGRSCSSFSATDLVELARETGWRVELSWARQYSQKGALDAVFHRHPVSAGSGRVMFQFPVETEDRPHISRTNRPLQRLQKKRTETHVHEQLRALLPRYMVPTRIVALDKLPVNANGKVDRQQLARTAQVLPASKAPSACVAPRNELEMTLCEEFSQVLGVEVGITDNFFHLGGHSLMATKLAARISRQLNIQVSVRDIFDYPVIVDLTDRLRLHHTRILTHDHGQHGQPDLKPFTLLPTNNPQEFLQHHILPQLVPDHAKILDVYPVTRIQRRFLHHPKRGLPRFPSMVFFDFPPGSDPHKLRLACMALVQRFDILRTIFLSVSGQFFQVVLDGYGIVIPVIEVDEELDDATRKLHDSDIQQPLRLGKPLIRIAVLKRQHSRVRAVLRLSHALYDGLSFEHIIQSLHALYLDITLSAPPKFGLYVQHMIQSRAEGYAFWRSVLKGSSMTILERSSTLQSRQPHLGRFLSAEKIIKAPLHANKSGITQATVFAAANALMLANLTGTNDVVFARIVSGRQSLPKNFQHVVGPCTNDVPVRVRMEPGVGPKALLRQVQDQYVHSFPFETLGFDEIKENCTDWPERITNFGCSTTYQNFDIFPKSQIDHQQIQMASLASEYQNRETWDEAPLYDLNVTGVPQPDGRHIKIYVGVDGQLCDESTLDCILSDICEGVVSLTDALQELPAASITE

SEQ ID NO: 7 - DNA, 2103 bp, Aureobasidium melanogenum strain W5-2
atggcttcatctaatggcccgatgaattccccctttgaattgatccccaaggtcgtcaataagaagaattactatactgacttcttgaagcgcgatgagcaattcctcgcatttcgccttcaaggcgaggagaaccgtaatcgcatgatcaaagctgcgcgcgataaggaccgcgcaatggctcaggctgcttctaatggagtctcagctgatgctgcgcaagctgagattgacgatgatgccgccgaggatgaagctgctgaagctgaagcctttggctcaaagacgattgtcattcatcctggcagtcgcaacctacgtattggtcttgcaacagacgcccttcccaagacaatcccgatggtgattgcacgcaaggcttcacatgcagaagacgaggagcctggcgctgaaccgcggccaaagcgagtcaagatgcaggatggtacggcagagcctgctggcgagagtgcgttcggcgaagatttcgcaaaggaatacagtagcatggcagctgacttcaaaatctaccgtcgcaacaacaaacgtagagtcttgcccaactcgcgtgaactggtcgtcaactggaactcgcgcaatgctccggaaaccatttctgaacataacgatcctcagcgtgttgactggacagaaattgtgtcacctgcacccgaaatcttcactggacatgcagctctgcgaataccacagcattccaaaccccgatacagactctactggccactcaaatgtggttggctcaatgaacaagactattcgagcaaatctagcttatttcgcgacttcttcagcatcatcgaagaggccatcaagaacgagcttcacctgaaccgtaagagagactgggcacagtactcttgcgtgttcatcattcccgatctgtacgagaaagttttcgtgacatccatcctcgaggaaatgttcagagacttcggtttccagcgtgtttgcttcatccaagaaagtctggcagcaacctttggagctggatactcgagcagttgtattgttgatgttggtgcacaaaagacttctatctgctgcgttgaggaaggcatgtgcgtcgagaactcccgcatgaacctgaagtttggcggagaagatgttacagaaacattcatcaagatgatgctgtacgaccacttcaattatgccaacatggatctgctgaggagacatgactaccttcttgcggaagagctgaagcaaaagttctgcacgctcgaggatgcacatatcagcgtacagctttatgagttccatctccgtgcgttcggccaagacactcgcaaataccagttcaagacgtatgatgaagtcatgctggcacctatgggtttcttcaggccaacaatatttgatcattcagacaagctcgctggcagacgcaagctcatcggtcgctcaactgacacttacgatgataaacctaatgatcccatgtcactcgctcaactgcaggtctacaagtactcgtccgataatgttccctcagctgtagcagaatcaagtacaccggcacctggtggcgtgcctgcaacacccagcaaacccttgaacctggaccgcctaacgcatcttgccgatgtagcggaaagtacacctcgttcctctccagcaggatcgcctgctcctgacgacacggcaacaccagtaccaggagctggagacgcaacaccagccgtagcaggtggcgggatcgaaggtgcacagccaaatactgaagatgtgctgcctgtgatgcccttggatcaagcaatcgtcacatgcatcaccgaaggcgccaagggtgatgagaagaagacgcgtgacttcttcggtggtatcatggtgatcggaggcggtagcaagacttacaatttcaacgtctatctcgagcagagacttcgcgcgctacagccaaacttccagaaggaaatcttggttggacctccgcctagagagctcgatcctcaggttctggtgtggaagggcggtagtgtgtttggcaagatgagaggcactaatgacagctggatcggacagttggagtttgacagactgggtgccagaatcttgaaccagaagtgtatgtgggcatac

SEQ ID NO: 8 - DNA, 1377 bp, Aureobasidium melanogenum strain W5-2
atgggtaaggaaaagtcccacattaacgtcgtcgttatcggccacgtcgactccggtaagtcgaccaccaccggtcacttgatctacaagtgcggtggtatcgacaagcgtaccatcgagaagttcgagaaggaagccgccgaactcggcaagggttccttcaagtacgcctgggtcctcgacaagctgaagtctgagcgtgagcgtggtatcactatcgatatcgccctgtggaagttcgagacccccaagtacatggtcaccgtcatcgacgcccccggtcaccgtgatttcatcaagaacatgatcactggtacctcgcaggctgactgcgccattctcatcattgccgccggtactggtgagttcgaggctggtatctccaaggatggccagacccgtgagcacgcccttctcgcctacaccctcggtgtcaagcagctcatcgttgccatcaacaagatggacaccaccaagtggtccgaggcccgttaccaggagatcatcaaggagacctccggtttcatcaagaaggtcggctacaaccccaagcacgttcccttcgtccccatctccggtttcaacggtgacaacatgatcgaggtttccaccaactgcccctggtacaagggttgggagaaggagaccaaggccaaggccaccggcaagactctcctcgaagccattgacgccatcgaccctcctacccgccccaccgacaagcccctccgtcttcccctccaggatgtctacaagatcggtggtattggcacggtgcccgtcggccgtgtcgagaccggtaccatcaagggtggtatggtcgtcaccttcgcccccgctggtgtcaccactgaggtcaagtccgtcgagatgcaccacgagcagctcgccgagggtcttcccggtgacaacgtcggcttcaacgtcaagaacgtctccgtcaaggagatccgtcgtggtaacgttgccggtgactccaagaacgacccccccaagggttgtgactccttcaacgcccaggtcatcgtcctgaaccaccccggtcaggtcggtgctggttacgcacccgtcctcgactgccacactgcccacatcgcctgcaagttctccgagcttgttgagaagatcgaccgccgtaccggcaagtccgttgaggccgcccccaagttcatcaagtctggtgacgccgccattgtcaagatggttccctccaagcccatgtgtgttgaggccttcactgactaccctcctctcggtcgtttcgccgtccgtgacatgagacagaccgtcgccgtcggtgtcatcaagtctgtcgccaagtccgacaagggtggtgccggtaaggtcactaaggccgccgtcaaggctggcaagaag

SEQ ID NO: 9 - DNA, 1341 bp, Aureobasidium melanogenum strain W5-2
atgcgtgagattgtccacctccagaccggccaatgcggtaaccaagttggtgctgccttctggcagaccatctctggcgagcacggccttgacggtgctggtgtctacaacggtacctcagatctccagctggagcgcatgaacgtctacttcaacgaggcctctggtaacaaatatgttccccgtgccgtcctcgtcgacttggagcctggtaccatggacgccgtccgtgctggtcctttcggtcagctcttccgtcccgacaacttcgtcttcggtcagtccggtgctggcaacaactgggccaagggtcactacactgagggtgccgagttggtcgaccaggtcttggatgtcgttcgtcgtgaggccgagagctgtgactgcctccaaggtttccagatcactcactcgctcggtggtggtaccggtgccggtatgggaacgctcctcatctccaagatccgtgaggagttccccgaccgtatgatggccaccttctccgtcatgccctcccccaaggtctccgacaccgttgtcgagccttacaacgctaccctctccgtccaccagctggtcgagaactctgacgagaccttctgtatcgacaaccaggctctctacgacatctgcatgagcaccctcaagctcaacaacccctcctacggcgacctgaactacctcgtctccgccgtcatgtccggtgttaccgtctcgctccgtttccctggccagctcaactccgacttgcgcaagctcgccgtcaacatggtccccttcccccgtctccacttcttcatggtcggttttgctcctctcaccagccgtaacgcccactcgttccgcgccgtctcggttcccgagctcacccagcaaatcttcgaccccaagaacatgatggccgccaccgatttccgcaacggccgctacctgacctgctctgccatcttccgtggtaaggtctccatgaaggaggtcgaggaccagatgcgcaacgtccagaacaagaactccgcctacttcgttgagtggatccccaacaacgtccagaccgccctctgctccattcctcctcgtggtcttaagatgtcatcgaccttcgtcggtaactcgacctcgatccaggagctgttcaagcgtgtcggtgaccagttctctgccatgttccgtcgcaaggctttcttgcactggtacactggtgagggtatggacgagatggagttcactgaggctgagtctaacatgaacgacttggtcagcgagtaccagcagtaccaggaggcttccatctccgagggtgaggaggagtacgacgaggaggctcctatggaggctgaggag

SEQ ID NO: 10 - DNA, 6093 bp, Aureobasidium melanogenum strain W5-2
cggccggcgccttgcaacatcaacgcccgtcatatcctcgacctcacccttgctgctaccacgccctcaccaaccgcatcgccgcgcatcacctccattgcgcgcaatcgccgtctcgagtcgcgtcgctccttcatcgcctgtcgatttctctgtttcgccgctgtccgcctgcgcgcgcgccgttcgaaaggccagtcgctcgacacgcgctcttccgccagaggcaaccctcttacatccacaatcatccaccttatcaccactttcatctgtcctggagatccacgctcaacctctccgtcgacagcgccctgaaggcggcagccgctgatacgattcttacacaatttctcttagctattgctatcaacatccgccaccatgaacatccactcttttccctattccagcgctccgctgaagaccattcaggagattcagtttggtctcttctctcctgaggagatcaagaacatgagtgtgtgtcacatcgagtacccagagaccatggacgagcaacggatgcgtccgcgagagaagggcttaaacgaccccaagctgggctctatcgatcgctcagttgcctgtggtacctgcggtgaagacatgctggagtgtcccggtcactttggtcatattgagcttgctgtgcccgtcttccacgtcggttttgtcaccaagatcaagaagattctcgaaaccgtctgccacaactgtggcaaagtcttgcttgatgaaagcattcctgccttcgcccaagctgtccgcataagagatcccaagcgccgcttcgatgctgttcacagactgtgcaaggccaagacgacctgcgatcccgatgaggctggtgacgatggagaagacccgaaagacgccttgaagaagggcaagcgatcacacggtggctgcggtaacctgcaacccacaattcgcaaggacggtcttaagcttaccggcacctacacataccccaaggacgccgatacagaacaaaagcccgtggagaagaaggtcatcacccctcagatggcactgaacgttttccgcaacatttcgacatacgacttggccagaatgggcctcaacgcagactacgctcgtcccgaatggatgatcctgaccgtgttgcccgtaccgccaccagctgttcgtcccagtgtttcggtcgatggaaccaaccaaggaatgcgttccgaggatgatttgactttcaaactcagtgatattatccgcgccaatgccaacgttcgcaagtgtgagctcgagggctctccacaccacgttattgcagagtttgaggctttgctgcagttccacgtcgctacatacatggacaacgatattgcaggacagcctaaggctctgcaaaaatccggtagacctgtcaaggctattcgtgcgcgcctgaagtccaaggagggtcgtcttcgtggtaaccttatgggcaagcgtgtcgatttctccgctcgtacagtcatcactggtgacccgaacttgtctctggatgaagtaggtgttcctagaagtaccgcccgcatccttaccttccccgagaccgtcaacgctttcaacatcgacaagctacaacaactcgtccgcaacggtcccaacgaacaccctggagcaaagtatgtcattcgagacactggcgagcgcatcgatttgcgccatcacaagcgcgctggcgagattcaactgcaatatggctacaaagtcgaaagacatatcgtcgatggtgatgttattatcttcaaccgtcaaccttcgctgcacaaggagtctatgatgggtcacagagtccgtgtcatgccctactctactttccgtctcaacctttccgttacttcgccatacaacgccgatttcgatggtgatgagatgaacttgcacgttcctcagagtcacgaaactcgctcagaagtcatgaacctttgcatggttcccctcaacatcgtctctcctcagcgtaacggtcccttgatgggtatcgtgcaagacactctttgtggtatctacaagatgtgccgtcgtgatgttttcctggaccaggaacacgtcatgaacattctcatgtgggtgcctgattgggacggtgtcatcccaccaccttctatcctcaaacctcgccctagatggactggtaagcagattatcagcttgatcgtccccactggtttgaaccttgttcgtggtgatgctgagggcatgcatcccctcaacgacaacggtttgatggtacatggtggcgagctcatgtacggtctgttcagcaagaagtccgtcggtgccagtggaggtggtatcatccacatcgtctacaacgaaaagggctgggaagctgctgtcagtttcttcaacggagctcagcgtgtcgtcaactactggctgctccacaacggtttcagtatcggtattggtgacacagttcctgacgaggcgactgccgaggccatcacagacgcagtcaatgagcagaaggcagaagtagctgtcatcaccgaggctgctactgctaacgagcttgaagctctgcctggtatgaacgttcgtgagacgttcgagagcagagtgtccaaggctttgaacagtgctcgtgacaacgctggtgaccgtacggaaaagagtttgaaggatttgaacaacgccattcagatggctcgttcaggttccaagggttcggctatcaacatttcgcagatgaccgctgtcgtcggccaacaatccgtcgagggaaagcgtattcctttcggcttcaagtacagatcgcttccccacttcaccaaggacgattactctcccgagtctcgtggtttcgtcgagaactcctatctccgcggattgacaccttcagaattcttcttccacgccatggctggtcgtgagggtctgatcgatactgctgtcaagactgccgaaactggttacattcagcgtcgtctcgtcaaggctcttgaagaagtcatggccaagtatgatggcactgttcgtaactccttgggcgatatcgtgcaattcgtctacggtgaagatggtttggatgctgtgcatatcgaaggtcaaaagttggatatcatcaactgctccgacagtcaattcgagaagaagttccgtattgatgtcatggaccccaagatgtctctttcacccgacattctcgagcaagcacacgagattgctggagatgttgaggtccagcgtcacctcgacgctgagtatgaagcattgttggctgacagagctctgctcagagatggccgtaccgatgacgaagaaacccaccaacttcctcttaacatcacccgtatcgtcgagagtgctaagaccagattccgcatcaaggatggcgctcgcagtgatcttcacccgtccgacgttattcccaaggttcagaacttgcttgaccagattgttgttgttcgtggtgacgaccctctttcccaagaagcacaatacaacgccactatcctcttcaaggccctgctcagatcacgtctcgcttttaagcgtctggtcaaggagtactctttgaacaagctcgcgcttgacaacattcttggtgatattctgaacagattctcaagatcgcttgtcagtcccggtgaaatggttggtgtcttggccgcacagtctattggagaacccgcaacacagatgacgctcaacactttccatttcgctggtgtctcgtccaagaacgttaccctcggtgtgccccgtctgaaggaaattctgaacgttgctaccaacatcaagacaccttccatgactgtctaccaatctgccgaaaaccgccttgatcaggaagcttgcaagcgacttcgtagtctggttgagtacaccagtttgcgctccattactgagaagaccgaaatttggttcgaccctgacattcaatcaaccgttgttgaacaagacagggatatggtcgagtcttacttcatcatccccgaagagaatgcagagagtcccgagacttactccaagtggttgctgcgtatcgttcttggtcgtagacagcttttggacaagggtctttcggtcgctgatgtcgccgctgctatcaagaatgtctaccaccaggagatgtctattatcttcagtgacgacaacgctgatgagcttgttattcgtatcagaccttcgaacgtgcttatggagtccaaagaagacgatgataccgctcttgaggccgatctgatcatcggaagactcgaaactcatctgttggacgagaccagacttcgtggtgtcttgggcgtcgatcgtgctttcgtcaacttcaaggaacgtctgcgcgtcaaggaagacggtgctcttactatgtccaagagcgatcctctttgcaaggaatggttcttggataccagcggaactgctctcaaggaagttcttactgttgagggcactgatcctacccgcacttacactaaccacttcattgacatcttcagtgtgttcggtattgaggctactagatccgcattgatgagagaactcaagcaagtgctttcgttcgacggttcttatgtcaaccatcgccatcttgccctcctggtcgatattatgaccgctcgcggtaaccttatggctgtcacccgtcacggtatcaaccgtgctgacactggtgcactgatgcgttgttcgttcgaagagacggtcgagattctgttcgaagctgcctcctcaggtgaacttgacgactgccgtggtgtttccgaaaacatcattcttggtcagcttgcaccttcgggtactggtgagtttgatgttcttttggaccagcagatgctcagcactgttgtctctcgtcaccatggtatgggtgctggtactcaagctggcgccgctcctcttgacggtgctatgactccctacgatatgggctctcctcttgccgagggcgactacggtactgcggactatggtgcttccttctctcctatggtccaggcaggtggcgacgagatgggtggtttctctgcctaccaaggtggaagcttcagcccttacagtggcggtcagagccctggttacgcacctaccagtccattcagcatgggtacaagcccatcatctcccggatatgcctcgccatcttctcctggctattcacccagatcacctggtgcagctcttggcagccccggctacggcatgggttcacctgccagtccggcgtacaacccaacatcgcccacttactcgcctacatctcctgcctacggcaagggctctcccacctcaccttcttactctcctacatctcccagctattcgccaacttcacccagctactcgcctacgtcgcctagctactctcctacctctccttcatacagccccacttctcctgctcacagaggatcgggcatttctccaacctctccacgatacagcccgacatctccggcttactcgcccacttcacctgcatacagcccgaccagcccctcctacaaccctggcggagcctcgcactcgcctacgtcgcccagctacagcccgacgtcgccagtgtacagcccaaccagtccggcacagcagggctattctcctacctcaccacagtacactcccaactctcctggtcaagcttcgcctaagtattcacctactagccccaagtactcgcccaactcgcctggccaataagcgaatgaagcgagcagttacccaactgggacgtaccctttgctgggcccacgtcttgtcatgggctagggttaatatcaaggtcaccaacattccgaaacaactcgtagtctgggttttggttcacgaagacgatgcacgagcgataagagcacaagcaggtacattgcgggagattttacaaggcgttcttctttttctttttctgctagtcttgtttttgagagaaggaaagttctccaaggtttgtttttcaggctcacaaaattgcatatggagaacgagccaagtgtagtatcagagaggatttttcgaggcaaagataaaccaaagatgagataacacaaatgcgaacaagcaagtccaaatttctgctttcgttgaaagtgactgctggccgagggcaaaaagcaagtgtaatatttttttatgtagtcg